European Patent Specification EP 4 370 687 B1, published April 9, 2025. Title: NEW SYSTEMS FOR PRODUCING RECOMBINANT PROTEINS/ NUOVI SISTEMI DI PRODUZIONE DI PROTEINE RICOMBINANTI. Applicant: NEMYSIS LIMITED. The sequence listing filed with the application follows.

SEQUENCE LISTING (30 sequences)

SEQ ID NO: 1 - protein, 325 aa, Actinoallomurus
  E40mat
AAPSGLSPANLQSAYKLPSSTAGSGQTVAIVDAYDAPTAEADLNVYRSQFGLGACTTANGCFKKVDQNGGTSYPRKDGGWAQEISLDLDMVSAVCPNCKIVLVEAKTNSFANLGTAENTAASLANVISNSYGGSDASDASYGSYYNHPGKAITVSSGDAGYGVEYPASSHYVTAVGGTSLRTASTSRGWSETAWSGAGSGCSAYNTALSGQSGLTGCSRRAVADVSAVADPATGVAVYDSTAYQGQSGWMVFGGTSVAAPIIGGVYGLAANAASIDNNYPYAHTSSLFDVTSGSNGTCTTTKWCTAGTGWDGPTGLGTPNGTGAF

SEQ ID NO: 2 - protein, 332 aa, Actinoallomurus
  E40 His mat
AAPSGLSPANLQSAYKLPSSTAGSGQTVAIVDAYDAPTAEADLNVYRSQFGLGACTTANGCFKKVDQNGGTSYPRKDGGWAQEISLDLDMVSAVCPNCKIVLVEAKTNSFANLGTAENTAASLANVISNSYGGSDASDASYGSYYNHPGKAITVSSGDAGYGVEYPASSHYVTAVGGTSLRTASTSRGWSETAWSGAGSGCSAYNTALSGQSGLTGCSRRAVADVSAVADPATGVAVYDSTAYQGQSGWMVFGGTSVAAPIIGGVYGLAANAASIDNNYPYAHTSSLFDVTSGSNGTCTTTKWCTAGTGWDGPTGLGTPNGTGAFGHHHHHH

SEQ ID NO: 3 - protein, 398 aa, Actinoallomurus
  E40 pre-pro
MSRRVTGTILGGLILAMVPFLSTAANAAPQAAPASVSHPFHHSCATVKPGRASCNALVRSDIAQSAATLAHQAAAPSGLSPANLQSAYKLPSSTAGSGQTVAIVDAYDAPTAEADLNVYRSQFGLGACTTANGCFKKVDQNGGTSYPRKDGGWAQEISLDLDMVSAVCPNCKIVLVEAKTNSFANLGTAENTAASLANVISNSYGGSDASDASYGSYYNHPGKAITVSSGDAGYGVEYPASSHYVTAVGGTSLRTASTSRGWSETAWSGAGSGCSAYNTALSGQSGLTGCSRRAVADVSAVADPATGVAVYDSTAYQGQSGWMVFGGTSVAAPIIGGVYGLAANAASIDNNYPYAHTSSLFDVTSGSNGTCTTTKWCTAGTGWDGPTGLGTPNGTGAF

SEQ ID NO: 4 - protein, 405 aa, Actinoallomurus
  E40 pre-pro His
MSRRVTGTILGGLILAMVPFLSTAANAAPQAAPASVSHPFHHSCATVKPGRASCNALVRSDIAQSAATLAHQAAAPSGLSPANLQSAYKLPSSTAGSGQTVAIVDAYDAPTAEADLNVYRSQFGLGACTTANGCFKKVDQNGGTSYPRKDGGWAQEISLDLDMVSAVCPNCKIVLVEAKTNSFANLGTAENTAASLANVISNSYGGSDASDASYGSYYNHPGKAITVSSGDAGYGVEYPASSHYVTAVGGTSLRTASTSRGWSETAWSGAGSGCSAYNTALSGQSGLTGCSRRAVADVSAVADPATGVAVYDSTAYQGQSGWMVFGGTSVAAPIIGGVYGLAANAASIDNNYPYAHTSSLFDVTSGSNGTCTTTKWCTAGTGWDGPTGLGTPNGTGAFGHHHHHH

SEQ ID NO: 5 - DNA, 1197 bp, Actinoallomurus
  E40 pre-pro
atgtcacgacgcgtgaccgggaccatactgggcgggttgatcctcgccatggtccccttcctttccaccgcggccaacgccgcaccccaggccgcgccggcttccgtctcccacccgttccaccactcctgcgccacggtgaagccgggtcgggcgagctgcaatgccctcgtacgcagcgacatcgcccagagcgcggcgaccctcgcgcaccaagcggccgccccatccgggctctcgccggccaacctgcagagcgcctacaagctgccgtcctccacggccggatccggccagaccgtcgcgatcgtcgacgcctatgacgccccgaccgccgaagcggacttgaacgtgtaccgaagccagttcggactcggcgcgtgcacgaccgccaacggctgtttcaagaaggtcgaccagaacggcggcacgtcctatccgaggaaggacggcggctgggcgcaggagatctccctggacctcgacatggtctccgcggtctgccccaactgcaagatcgttctcgtcgaggcgaagaccaactcgttcgccaacctgggtaccgccgagaacaccgcggcgagtctcgcgaacgtcatcagcaacagctacggcggctcggacgcctctgacgcgagctatggctcgtactacaaccacccgggcaaggccatcacggtcagctccggcgacgccggctacggcgtggagtacccggcctcgtcccactacgtgaccgccgtcggcggcacctcgctgcgcaccgcgagcaccagccgcggctggagcgagaccgcgtggagcggcgcgggcagtggctgctcggcctacaacaccgcgctgtccggccagtccggcctcaccggctgctcccggcgcgccgtcgccgacgtctccgccgtggccgacccggccaccggcgtcgccgtctacgacagcacggcctaccagggccagagcggctggatggtcttcggcggcaccagcgtcgccgcaccgatcatcggtggcgtgtacggcctcgccgccaacgccgcgagcatcgacaacaactacccctacgcccacaccagctcgctcttcgacgtcacgtcgggcagcaacggcacctgcaccaccaccaagtggtgcaccgccggcaccggctgggacggccccaccggcctcggaacgccgaacggcaccggagccttctga

SEQ ID NO: 6 - DNA, 1218 bp, Actinoallomurus
  E40 pre-pro His
atgtcacgacgcgtgaccgggaccatactgggcgggttgatcctcgccatggtccccttcctttccaccgcggccaacgccgcaccccaggccgcgccggcttccgtctcccacccgttccaccactcctgcgccacggtgaagccgggtcgggcgagctgcaatgccctcgtacgcagcgacatcgcccagagcgcggcgaccctcgcgcaccaagcggccgccccatccgggctctcgccggccaacctgcagagcgcctacaagctgccgtcctccacggccggatccggccagaccgtcgcgatcgtcgacgcctatgacgccccgaccgccgaagcggacttgaacgtgtaccgaagccagttcggactcggcgcgtgcacgaccgccaacggctgtttcaagaaggtcgaccagaacggcggcacgtcctatccgaggaaggacggcggctgggcgcaggagatctccctggacctcgacatggtctccgcggtctgccccaactgcaagatcgttctcgtcgaggcgaagaccaactcgttcgccaacctgggtaccgccgagaacaccgcggcgagtctcgcgaacgtcatcagcaacagctacggcggctcggacgcctctgacgcgagctatggctcgtactacaaccacccgggcaaggccatcacggtcagctccggcgacgccggctacggcgtggagtacccggcctcgtcccactacgtgaccgccgtcggcggcacctcgctgcgcaccgcgagcaccagccgcggctggagcgagaccgcgtggagcggcgcgggcagtggctgctcggcctacaacaccgcgctgtccggccagtccggcctcaccggctgctcccggcgcgccgtcgccgacgtctccgccgtggccgacccggccaccggcgtcgccgtctacgacagcacggcctaccagggccagagcggctggatggtcttcggcggcaccagcgtcgccgcaccgatcatcggtggcgtgtacggcctcgccgccaacgccgcgagcatcgacaacaactacccctacgcccacaccagctcgctcttcgacgtcacgtcgggcagcaacggcacctgcaccaccaccaagtggtgcaccgccggcaccggctgggacggccccaccggcctcggaacgccgaacggcaccggagccttcggacaccaccaccaccaccactga

SEQ ID NO: 7 - DNA, 5789 bp, plasmid pIJ86
  pIJ86
  unsure 2579..2582: /note="n can be any of A, T, G, C"
gccagcctcgcagagcaggattcccgttgagcaccgccaggtgcgaataagggacagtgaagaaggaacacccgctcgcgggtgggcctacttcacctatcctgcccggctgacgccgttggatacaccaaggaaagtctacacgaaccctttggcaaaatcctgtatatcgtgcgaaaaaggatggatataccgaaaaaatcgctataatgaccccgaagcagggttatgcagcggaaaagatccgtcgacctgcaggtcgactctagaggatctggggaattcgagctcggtaccagcccgacccgagcacgcgccggcacgcctggtcgatgtcggaccggagttcgaggtacgcggcttgcaggtccaggaaggggacgtccatgcgagtgtccgttcgagtggcggcttgcgcccgatgctagtcgcggttgatcggcgatcgcaggtgcacgcggtcgatcttgacggctggcgagaggtgcggggaggatctgaccgacgcggtccacacgtggcaccgcgatgctgttgtgggcacaatcgtgccggttggtaggatcctctagagtcgaccggcatgcaagcttggctgcagatctgatccgcggggcgccggcacttcgtgctggcgccccgcccccacccaccaggagaccgaccatgaccgacttcgacggacgcctgaccgaggggaccgtgaacctggtccaggaccccaacggcggtggctggtccgcccactgcgctgagcccggttgcgactgggccgacttcgccggaccgctcggcttccagggcctcgtggccatcgctcgccgacacacgcactgaccgcacgtcaaagccccgccggatcaccggcggggctctcttcggccctccaagtcacaccagccccaaggggcgtcgggagtggcggagggaacctctggcccgattggtgccaggattcccaccagaccaaagagcaacgggccggacttcgcacctccgacccgtccgctcccagactcgcgccccttagccgggcgagacaggaacgttgctcgtgcccagagtacggagcgatgccgaggcattgccagatcggcccgccgggccccgctgccactgcgggaccgcaattgcccacacaccgggcaaacggccgcgtatctactgctcagaccgctgccggatggcagcgaagcgggcgatcgcgcgtgtgacgcgagatgccgcccgaggcaaaagcgaacaccttgggaaagaaacaacagagtttcccgcacccctccgacctgcggtttctccggacggggtggatggggagagcccgagaggcgacagcctctgggaagtaggaagcacgtcgcggaccgaggctgcccgactgcggaaagccgcccggtacagccgccgccggacgctgtggcggatcagcggggacgccgcgtgcaagggctgcggccgcgccctgatggaccctgcctccggcgtgatcgtcgcccagacggcggccggaacgtccgtggtcctgggcctgatgcggtgcgggcggatctggctctgcccggtctgcgccgccacgatccggcacaagcgggccgaggagatcaccgccgccgtggtcgagtggatcaagcgcggggggaccgcctacctggtcaccttcacggcccgccatgggcacacggaccggctcgcggacctcatggacgccctccagggcacccggaagacgccggacagcccccggcggccgggcgcctaccagcgactgatcacgggcggcacgtgggccggacgccgggccaaggacgggcaccgggccgccgaccgcgagggcatccgagaccggatcgggtacgtcggcatgatccgcgcgaccgaagtcaccgtggggcagatcaacggctggcacccgcacatccacgcgatcgtcctggtcggcggccggaccgagggggagcggtccgcgaagcagatcgtcgccaccttcgagccgaccggcgccgcgctcgacgagtggcaggggcactggcggtccgtgtggaccgccgccctgcgcaaggtcaaccccgccttcacgcccgacgaccggcacggcgtcgacttcaagcggctggagaccgagcgcgacgccaacgacctcgccgagtacatcgccaagacccaggacgggaaggcgcccgccctcgaactcgcccgcgccgacctcaagacggcgaccggcgggaacgtcgccccgttcgaactcctcggacggatcggggacctgaccggcggcatgaccgaggacgacgccgccggggtcggctcgctggagtggaacctctcgcgctggcacgagtacgagcgggcaacccggggacgccgggccatcgaatggacccgctacctgcggcagatgctcgggctcgacggcggcgacaccgaggccgacgacctcgatctgctcctggcggccgacgccgacggcggggagctgcgggccggggtcgccgtgaccgaggacggatggcacgcggtcacccgccgcgccctcgacctcgaggcgacccgggccgccgaaggcaaggacggcaacgagnnnncggcggccgtgggcgaacgggtgcgggaggtcctggcgctggccgacgcggccgacacagtggtggtgctcacggcgggggaggtggccgaggcgtacgccgacatgctcgccgccctcgcccagcgccgcgaggaagcaactgcacgccgacggcgagagcaggacgacgaccaggacgacgacgccgacgaccgccaggagcgggccgcccggcacatcgcccggctcgcaagtgggcccacttcgcactaactcgctcccccccgccgtacgtcatcccggtgacgtacggcgggggtcggtgacgtacgcggcgacggcggccggggtcgaagccgcggccgcgcgcgatatcgaattcgtaatcatggtcatagctgtttcctgtgtgaaattgttatccgctcacaattccacacaacatacgagccggaagcataaagtgtaaagcctggggtgcctaatgagtgagctaactcacattaattgcgttgcgctcactgcccgctttccagtcgggaaacctgtcgtgccagctgcattaatgaatcggccaacgcgcggggagaggcggtttgcgtattgggcgctcttccgcttcctcgctcactgactcgctgcgctcggtcgttcggctgcggcgagcggtatcagctcactcaaaggcggtaatacggttatccacagaatcaggggataacgcaggaaagaacatgtgagcaaaaggccagcaaaaggccaggaaccgtaaaaaggccgcgttgctggcgtttttccataggctccgcccccctgacgagcatcacaaaaatcgacgctcaagtcagaggtggcgaaacccgacaggactataaagataccaggcgtttccccctggaagctccctcgtgcgctctcctgttccgaccctgccgcttaccggatacctgtccgcctttctcccttcgggaagcgtggcgctttctcatagctcacgctgtaggtatctcagttcggtgtaggtcgttcgctccaagctgggctgtgtgcacgaaccccccgttcagcccgaccgctgcgccttatccggtaactatcgtcttgagtccaacccggtaagacacgacttatcgccactggcagcagccactggtaacaggattagcagagcgaggtatgtaggcggtgctacagagttcttgaagtggtggcctaactacggctacactagaagaacagtatttggtatctgcgctctgctgaagccagttaccttcggaaaaagagttggtagctcttgatccggcaaacaaaccaccgctggtagcggtggtttttttgtttgcaagcagcagattacgcgcagaaaaaaaggatctcaagaagatcctttgatcttttctacggggtctgacgctcagtggaacgaaaactcacgttaagggattttggtcatgagattatcaaaaaggatcttcacctagatccttttggttcatgtgcagctccatcagcaaaaggggatgataagtttatcaccaccgactatttgcaacagcgccggtgatcgtgctatgatcgactgatgtcatcagcggtggagtgcaatgtcgtgcaatacgaatggcgaaaagccgagctcatcggtcagcttctcaaccttggggttacccccggcggtgtgctgctggtccacagctccttccgtagcgtccggcccctcgaagatgggccacttggactgatcgaggccctgcgtgctgcgctgggtccgggagggacgctcgtcatgccctcgtggtcaggtctggacgacgagccgttcgatcctgccacgtcgcccgttacaccggaccttggagttgtctctgacacattctggcgcctgccaaatgtaaagcgcagcgcccatccatttgcctttgcggcagcggggccacaggcagagcagatcatctctgatccattgcccctgccacctcactcgcctgcaagcccggtcgcccgtgtccatgaactcgatgggcaggtacttctcctcggcgtgggacacgatgccaacacgacgctgcatcttgccgagttgatggcaaaggttccctatggggtgccgagacactgcaccattcttcaggatggcaagttggtacgcgtcgattatctcgagaatgaccactgctgtgagcgctttgccttggcggacaggtggctcaaggagaagagccttcagaaggaaggtccagtcggtcatgcctttgctcggttgatccgctcccgcgacattgtggcgacagccctgggtcaactgggccgagatccgttgatcttcctgcatccgccagaggcgggatgcgaagaatgcgatgccgctcgccagtcgattggctgagctcatgagcggagaacgagatgacgttggaggggcaaggtcgcgctgattgctggggcaacacgtggagcggatcggggattgtctttcttcagctcgctgatgatatgctgacgctcaatgccgtttggcctccgactaacgaaaatcccgcatttggacggctgatccgattggcacggcggacggcgaatggcggagcagacgctcgtccgggggcaatgagatatgaaaaagcctgaactcaccgcgacgtatcgggccctggccagctagctagagtcgacctgcaggtccccggggatcggtcttgccttgctcgtcggtgatgtacttcaccagcttcgcgaagtcgctcttcttgatggagcgcatggggacgtgcttggcaatcacgcgcaccccccggccgttttagcggctaaaaaagtcatggctctgccctcgggcggaccacgcccatcatgaccttgccaagctcgtcctgcttctcttcgatcttcgccagcagggcgaggatcgtggcatcaccgaaccgcgccgtgcgcgggtcgtcggtgagccagagtttcagcaggccgcccaggcggcccaggtcgccattgatgcgggccagctcgcggacgtgctcatagtccacgacgcccgtgattttgtagccctggccgacggccagcaggtaggccgacaggctcatgccggccgccgccgccttttcctcaatcgctcttcgttcgtctggaaggcagtacaccttgataggtgggctgcccttcctggttggcttggtttcatcagccatccgcttgccctcatctgttacgccggcggtagccg

SEQ ID NO: 8 - DNA, 6986 bp, plasmid pIJ86
  pIJ86 E40 His
  unsure 3776..3779: /note="n can be any of A, T, G, C"
gccagcctcgcagagcaggattcccgttgagcaccgccaggtgcgaataagggacagtgaagaaggaacacccgctcgcgggtgggcctacttcacctatcctgcccggctgacgccgttggatacaccaaggaaagtctacacgaaccctttggcaaaatcctgtatatcgtgcgaaaaaggatggatataccgaaaaaatcgctataatgaccccgaagcagggttatgcagcggaaaagatccgtcgacctgcaggtcgactctagaggatctggggaattcgagctcggtaccagcccgacccgagcacgcgccggcacgcctggtcgatgtcggaccggagttcgaggtacgcggcttgcaggtccaggaaggggacgtccatgcgagtgtccgttcgagtggcggcttgcgcccgatgctagtcgcggttgatcggcgatcgcaggtgcacgcggtcgatcttgacggctggcgagaggtgcggggaggatctgaccgacgcggtccacacgtggcaccgcgatgctgttgtgggcacaatcgtgccggttggtaggatcaatgtcacgacgcgtgaccgggaccatactgggcgggttgatcctcgccatggtccccttcctttccaccgcggccaacgccgcaccccaggccgcgccggcttccgtctcccacccgttccaccactcctgcgccacggtgaagccgggtcgggcgagctgcaatgccctcgtacgcagcgacatcgcccagagcgcggcgaccctcgcgcaccaagcggccgccccatccgggctctcgccggccaacctgcagagcgcctacaagctgccgtcctccacggccggatccggccagaccgtcgcgatcgtcgacgcctatgacgccccgaccgccgaagcggacttgaacgtgtaccgaagccagttcggactcggcgcgtgcacgaccgccaacggctgtttcaagaaggtcgaccagaacggcggcacgtcctatccgaggaaggacggcggctgggcgcaggagatctccctggacctcgacatggtctccgcggtctgccccaactgcaagatcgttctcgtcgaggcgaagaccaactcgttcgccaacctgggtaccgccgagaacaccgcggcgagtctcgcgaacgtcatcagcaacagctacggcggctcggacgcctctgacgcgagctatggctcgtactacaaccacccgggcaaggccatcacggtcagctccggcgacgccggctacggcgtggagtacccggcctcgtcccactacgtgaccgccgtcggcggcacctcgctgcgcaccgcgagcaccagccgcggctggagcgagaccgcgtggagcggcgcgggcagtggctgctcggcctacaacaccgcgctgtccggccagtccggcctcaccggctgctcccggcgcgccgtcgccgacgtctccgccgtggccgacccggccaccggcgtcgccgtctacgacagcacggcctaccagggccagagcggctggatggtcttcggcggcaccagcgtcgccgcaccgatcatcggtggcgtgtacggcctcgccgccaacgccgcgagcatcgacaacaactacccctacgcccacaccagctcgctcttcgacgtcacgtcgggcagcaacggcacctgcaccaccaccaagtggtgcaccgccggcaccggctgggacggccccaccggcctcggaacgccgaacggcaccggagccttcggacaccaccaccaccaccactgaagcttggctgcagatctgatccgcggggcgccggcacttcgtgctggcgccccgcccccacccaccaggagaccgaccatgaccgacttcgacggacgcctgaccgaggggaccgtgaacctggtccaggaccccaacggcggtggctggtccgcccactgcgctgagcccggttgcgactgggccgacttcgccggaccgctcggcttccagggcctcgtggccatcgctcgccgacacacgcactgaccgcacgtcaaagccccgccggatcaccggcggggctctcttcggccctccaagtcacaccagccccaaggggcgtcgggagtggcggagggaacctctggcccgattggtgccaggattcccaccagaccaaagagcaacgggccggacttcgcacctccgacccgtccgctcccagactcgcgccccttagccgggcgagacaggaacgttgctcgtgcccagagtacggagcgatgccgaggcattgccagatcggcccgccgggccccgctgccactgcgggaccgcaattgcccacacaccgggcaaacggccgcgtatctactgctcagaccgctgccggatggcagcgaagcgggcgatcgcgcgtgtgacgcgagatgccgcccgaggcaaaagcgaacaccttgggaaagaaacaacagagtttcccgcacccctccgacctgcggtttctccggacggggtggatggggagagcccgagaggcgacagcctctgggaagtaggaagcacgtcgcggaccgaggctgcccgactgcggaaagccgcccggtacagccgccgccggacgctgtggcggatcagcggggacgccgcgtgcaagggctgcggccgcgccctgatggaccctgcctccggcgtgatcgtcgcccagacggcggccggaacgtccgtggtcctgggcctgatgcggtgcgggcggatctggctctgcccggtctgcgccgccacgatccggcacaagcgggccgaggagatcaccgccgccgtggtcgagtggatcaagcgcggggggaccgcctacctggtcaccttcacggcccgccatgggcacacggaccggctcgcggacctcatggacgccctccagggcacccggaagacgccggacagcccccggcggccgggcgcctaccagcgactgatcacgggcggcacgtgggccggacgccgggccaaggacgggcaccgggccgccgaccgcgagggcatccgagaccggatcgggtacgtcggcatgatccgcgcgaccgaagtcaccgtggggcagatcaacggctggcacccgcacatccacgcgatcgtcctggtcggcggccggaccgagggggagcggtccgcgaagcagatcgtcgccaccttcgagccgaccggcgccgcgctcgacgagtggcaggggcactggcggtccgtgtggaccgccgccctgcgcaaggtcaaccccgccttcacgcccgacgaccggcacggcgtcgacttcaagcggctggagaccgagcgcgacgccaacgacctcgccgagtacatcgccaagacccaggacgggaaggcgcccgccctcgaactcgcccgcgccgacctcaagacggcgaccggcgggaacgtcgccccgttcgaactcctcggacggatcggggacctgaccggcggcatgaccgaggacgacgccgccggggtcggctcgctggagtggaacctctcgcgctggcacgagtacgagcgggcaacccggggacgccgggccatcgaatggacccgctacctgcggcagatgctcgggctcgacggcggcgacaccgaggccgacgacctcgatctgctcctggcggccgacgccgacggcggggagctgcgggccggggtcgccgtgaccgaggacggatggcacgcggtcacccgccgcgccctcgacctcgaggcgacccgggccgccgaaggcaaggacggcaacgagnnnncggcggccgtgggcgaacgggtgcgggaggtcctggcgctggccgacgcggccgacacagtggtggtgctcacggcgggggaggtggccgaggcgtacgccgacatgctcgccgccctcgcccagcgccgcgaggaagcaactgcacgccgacggcgagagcaggacgacgaccaggacgacgacgccgacgaccgccaggagcgggccgcccggcacatcgcccggctcgcaagtgggcccacttcgcactaactcgctcccccccgccgtacgtcatcccggtgacgtacggcgggggtcggtgacgtacgcggcgacggcggccggggtcgaagccgcggccgcgcgcgatatcgaattcgtaatcatggtcatagctgtttcctgtgtgaaattgttatccgctcacaattccacacaacatacgagccggaagcataaagtgtaaagcctggggtgcctaatgagtgagctaactcacattaattgcgttgcgctcactgcccgctttccagtcgggaaacctgtcgtgccagctgcattaatgaatcggccaacgcgcggggagaggcggtttgcgtattgggcgctcttccgcttcctcgctcactgactcgctgcgctcggtcgttcggctgcggcgagcggtatcagctcactcaaaggcggtaatacggttatccacagaatcaggggataacgcaggaaagaacatgtgagcaaaaggccagcaaaaggccaggaaccgtaaaaaggccgcgttgctggcgtttttccataggctccgcccccctgacgagcatcacaaaaatcgacgctcaagtcagaggtggcgaaacccgacaggactataaagataccaggcgtttccccctggaagctccctcgtgcgctctcctgttccgaccctgccgcttaccggatacctgtccgcctttctcccttcgggaagcgtggcgctttctcatagctcacgctgtaggtatctcagttcggtgtaggtcgttcgctccaagctgggctgtgtgcacgaaccccccgttcagcccgaccgctgcgccttatccggtaactatcgtcttgagtccaacccggtaagacacgacttatcgccactggcagcagccactggtaacaggattagcagagcgaggtatgtaggcggtgctacagagttcttgaagtggtggcctaactacggctacactagaagaacagtatttggtatctgcgctctgctgaagccagttaccttcggaaaaagagttggtagctcttgatccggcaaacaaaccaccgctggtagcggtggtttttttgtttgcaagcagcagattacgcgcagaaaaaaaggatctcaagaagatcctttgatcttttctacggggtctgacgctcagtggaacgaaaactcacgttaagggattttggtcatgagattatcaaaaaggatcttcacctagatccttttggttcatgtgcagctccatcagcaaaaggggatgataagtttatcaccaccgactatttgcaacagcgccggtgatcgtgctatgatcgactgatgtcatcagcggtggagtgcaatgtcgtgcaatacgaatggcgaaaagccgagctcatcggtcagcttctcaaccttggggttacccccggcggtgtgctgctggtccacagctccttccgtagcgtccggcccctcgaagatgggccacttggactgatcgaggccctgcgtgctgcgctgggtccgggagggacgctcgtcatgccctcgtggtcaggtctggacgacgagccgttcgatcctgccacgtcgcccgttacaccggaccttggagttgtctctgacacattctggcgcctgccaaatgtaaagcgcagcgcccatccatttgcctttgcggcagcggggccacaggcagagcagatcatctctgatccattgcccctgccacctcactcgcctgcaagcccggtcgcccgtgtccatgaactcgatgggcaggtacttctcctcggcgtgggacacgatgccaacacgacgctgcatcttgccgagttgatggcaaaggttccctatggggtgccgagacactgcaccattcttcaggatggcaagttggtacgcgtcgattatctcgagaatgaccactgctgtgagcgctttgccttggcggacaggtggctcaaggagaagagccttcagaaggaaggtccagtcggtcatgcctttgctcggttgatccgctcccgcgacattgtggcgacagccctgggtcaactgggccgagatccgttgatcttcctgcatccgccagaggcgggatgcgaagaatgcgatgccgctcgccagtcgattggctgagctcatgagcggagaacgagatgacgttggaggggcaaggtcgcgctgattgctggggcaacacgtggagcggatcggggattgtctttcttcagctcgctgatgatatgctgacgctcaatgccgtttggcctccgactaacgaaaatcccgcatttggacggctgatccgattggcacggcggacggcgaatggcggagcagacgctcgtccgggggcaatgagatatgaaaaagcctgaactcaccgcgacgtatcgggccctggccagctagctagagtcgacctgcaggtccccggggatcggtcttgccttgctcgtcggtgatgtacttcaccagcttcgcgaagtcgctcttcttgatggagcgcatggggacgtgcttggcaatcacgcgcaccccccggccgttttagcggctaaaaaagtcatggctctgccctcgggcggaccacgcccatcatgaccttgccaagctcgtcctgcttctcttcgatcttcgccagcagggcgaggatcgtggcatcaccgaaccgcgccgtgcgcgggtcgtcggtgagccagagtttcagcaggccgcccaggcggcccaggtcgccattgatgcgggccagctcgcggacgtgctcatagtccacgacgcccgtgattttgtagccctggccgacggccagcaggtaggccgacaggctcatgccggccgccgccgccttttcctcaatcgctcttcgttcgtctggaaggcagtacaccttgataggtgggctgcccttcctggttggcttggtttcatcagccatccgcttgccctcatctgttacgccggcggtagccg

SEQ ID NO: 9 - protein, 371 aa, Actinoallomurus
  E40 pre
APQAAPASVSHPFHHSCATVKPGRASCNALVRSDIAQSAATLAHQAAAPSGLSPANLQSAYKLPSSTAGSGQTVAIVDAYDAPTAEADLNVYRSQFGLGACTTANGCFKKVDQNGGTSYPRKDGGWAQEISLDLDMVSAVCPNCKIVLVEAKTNSFANLGTAENTAASLANVISNSYGGSDASDASYGSYYNHPGKAITVSSGDAGYGVEYPASSHYVTAVGGTSLRTASTSRGWSETAWSGAGSGCSAYNTALSGQSGLTGCSRRAVADVSAVADPATGVAVYDSTAYQGQSGWMVFGGTSVAAPIIGGVYGLAANAASIDNNYPYAHTSSLFDVTSGSNGTCTTTKWCTAGTGWDGPTGLGTPNGTGAF

SEQ ID NO: 10 - DNA, 47 bp, Unknown
  KasOp* promoter
gtctctgctttgacaacatgctgtgcggtgttgtaaagtctggtgta

SEQ ID NO: 11 - DNA, 20 bp, PhiC31-like viruses
  SR40 RBS
cttgtcaaaggagtgtccat

SEQ ID NO: 12 - DNA, 87 bp, Streptomyces venezuelae
  Vsi signal peptide
atgcgtcgcaccctcaaggccgtgggagcagccgcggcggcggccacctgcgtcctcgccgcgacggcaggcaccgcgcaggccgag

SEQ ID NO: 13 - DNA, 85 bp, Unknown
  attP; PhiBT1 integrase attachment site
tcagacgtttcgggtgctgggttgttgtctctggacagtgatccatgggaaactactcagcaccaccaatgttcccaaaagaaag

SEQ ID NO: 14 - DNA, 5697 bp, pMU1s
  pMU1s-kasOp
tggcgccggacggggcttcagacgtttcgggtgctgggttgttgtctctggacagtgatccatgggaaactactcagcaccaccaatgttcccaaaagaaagcgcaggtcagcgcccatgagccaagatctaggcatgtcgcccttcatcgctcccgacgtccctgagcaccttctagacactgttcgcgtcttcctgtacgcgcgtcagtctaagggccggtccgacggctcagacgtgtcgaccgaagcacagctagcggccggtcgtgcgttggtcgcgtctcgcaacgcccaggggggtgcgcgctgggtcgtggcaggtgagttcgtggacgtcgggcgctccggctgggacccgaacgtgacccgtgccgacttcgagcgcatgatgggcgaagtccgcgccggcgaaggtgacgttgtcgttgtgaatgagctttcccggctcactcgcaagggcgcccatgacgcgctcgaaatcgacaacgaattgaagaagcacggcgtgcgcttcatgtcggttcttgagccgttccttgacacgtctacccctatcggcgtcgccattttcgcgctgatcgctgcccttgcgaaacaggacagtgacctgaaggcggagcgcctgaagggtgcgaaagacgagattgccgcgctgggtggcgttcactcgtcttccgccccgttcggaatgcgcgccgtgcgcaagaaggtcgataatctcgtgatctccgttcttgagccggacgaagacaacccggatcacgtcgagctagttgagcgcatggcgaaaatgtcgttcgaaggcgtgtccgacaacgccattgcaacgaccttcgagaaggaaaagatcccgtcgcccggaatggctgagagacgcgccacggaaaagcgtcttgcgtccgtcaaggcacgtcgcctgaacggcgctgaaaagccgatcatgtggcgcgctcaaacggtccgatggattctcaaccatcccgcaatcggcggtttcgcattcgagcgtgtgaagcacggtaaggcgcacatcaacgtcatacggcgcgaccccggcggcaagccgctaacgccccacacgggcattctcagcggctcgaagtggcttgagcttcaagagaagcgttccgggaagaatctcagcgaccggaagcctggggccgaagtcgaaccgacgcttctgagcgggtggcgtttcctggggtgccgaatctgcggcggctcaatgggtcagtcccagggtggccgtaagcgcaacggcgaccttgccgaaggcaattacatgtgcgccaacccgaaggggcacggcggcttgtcggtcaagcgcagcgaactggacgaattcgttgcttcgaaggtgtgggcacggctccgcacagccgacatggaagatgaacacgatcaggcatggattgccgccgctgcggagcgcttcgcccttcagcacgacctagcgggggtggccgatgagcggcgcgaacaacaggcgcacctagacaacgtgcggcgctccatcaaggaccttcaggcggaccgtaagcccggtctgtacgtcgggcgtgaagagctggaaacgtggcgctcaacggtgctgcaataccggtcctacgaagcggagtgcacgacccgactcgctgagcttgacgagaagatgaacggcagcacccgcgttccgtctgagtggttcagcggcgaagacccgacggccgaagggggcatctgggcaagctgggacgtgtacgagcgtcgggagttcctgagcttcttccttgactccgtcatggtcgaccgggggcgccaccctgagacgaagaaatacatccccctgaaggaccgtgtgacgctcaagtgggcggagctgctgaaggaggaagacgaagcgagcgaagccactgagcgggagcttgcggcgctgtagcgcacagcgggaggggtcgagccggcggacggttcggccccttttttggccttgaaatcgttagttaggctaactagggtaccgtctctgctttgacaacatgctgtgcggtgttgtaaagtctggtgtaggagaatacgacagcttgtcaaaggagtgtccatatgggatccagatatcctgcaggaattcctcgagccgatatccctctagaccgcggccgcccggctgcagcccgtacctctagtagagtcgagggggaacccggccgcgtccggcgcccccgccgccttcgacgagatcccgcaaaagcggcctttgactccctgcaagcctcagcgaccgaatatatcggttatgcgtgggcgatggttgttgtcattgtcggcgcaactatcggtatcaagctgtttaagaaattcacctcgaaagcaagctgataaaccgatacaattaaaggctccttttggagcctttttttttggagattttcaacgtgaaaaaattattattcgcaattcctttagttgttcctttctattctcactccgctgaaactgttgaaagttgtttagcaaaacctcatacagaaaattcatttactaacgtctggaaagacgacaaaactttagatcctctagctagagtcgaccggcatgcaatcgaattcgtaatcatgtcatagctgtttcctgtgtgaaattgttatccgctcacaattccacacaacatacgagccggaagcataaagtgtaaagcctggggtgcctaatgagtgagctaactcacattaattgcgttgcgctcactgcccgctttccagtcgggaaacctgtcgtgccagctgcattaatgaatcggccaacgcgcggggagaggcggtttgcgtattgggcgctcttccgcttcctcgctcactgactcgctgcgctcggtcgttcggctgcggcgagcggtatcagctcactcaaaggcggtaatacggttatccacagaatcaggggataacgcaggaaagaacatgtgagcaaaaggccagcaaaaggccaggaaccgtaaaaaggccgcgttgctggcgtttttccataggctccgcccccctgacgagcatcacaaaaatcgacgctcaagtcagaggtggcgaaacccgacaggactataaagataccaggcgtttccccctggaagctccctcgtgcgctctcctgttccgaccctgccgcttaccggatacctgtccgcctttctcccttcgggaagcgtggcgctttctcatagctcacgctgtaggtatctcagttcggtgtaggtcgttcgctccaagctgggctgtgtgcacgaaccccccgttcagcccgaccgctgcgccttatccggtaactatcgtcttgagtccaacccggtaagacacgacttatcgccactggcagcagccactggtaacaggattagcagagcgaggtatgtaggcggtgctacagagttcttgaagtggtggcctaactacggctacactagaagaacagtatttggtatctgcgctctgctgaagccagttaccttcggaaaaagagttggtagctcttgatccggcaaacaaaccaccgctggtagcggtggtttttttgtttgcaagcagcagattacgcgcagaaaaaaaggatctcaagaagatcctttgatcttttctacggggtctgacgctcagtggaacgaaaactcacgttaagggattttggtcatgagattatcaaaaaggatcttcacctagatccttttggttcatgtgcagctccatcagcaaaaggggatgataagtttatcaccaccgactatttgcaacagtgccgttgatcgtgctatgatcgactgatgtcatcagcggtggagtgcaatgtcgtgcaatacgaatggcgaaaagccgagctcatcggtcagcttctcaaccttggggttacccccggcggtgtgctgctggtccacagctccttccgtagcgtccggcccctcgaagatgggccacttggactgatcgaggccctgcgtgctgcgctgggtccgggagggacgctcgtcatgccctcgtggtcaggtctggacgacgagccgttcgatcctgccacgtcgcccgttacaccggaccttggagttgtctctgacacattctggcgcctgccaaatgtaaagcgcagcgcccatccatttgcctttgcggcagcggggccacaggcagagcagatcatctctgatccattgcccctgccacctcactcgcctgcaagcccggtcgcccgtgtccatgaactcgatgggcaggtacttctcctcggcgtgggacacgatgccaacacgacgctgcatcttgccgagttgatggcaaaggttccctatggggtgccgagacactgcaccattcttcaggatggcaagttggtacgcgtcgattatctcgagaatgaccactgctgtgagcgctttgccttggcggacaggtggctcaaggagaagagccttcagaaggaaggtccagtcggtcatgcctttgctcggttgatccgctcccgcgacattgtggcgacagccctgggtcaactgggccgagatccgttgatcttcctgcatccgccagaggcgggatgcgaagaatgcgatgccgctcgccagtcgattggctgagctcatgagcggagaacgagatgacgttggaggggcaaggtcgcgctgattgctggggcaacacgtggagcggatcggggattgtctttcttcagctcgctgatgatatgctgacgctcaatgccgtttggcctccgactaacgaaaatcccgcatttggacggctgatccgattggcacggcggacggcgaatggcggagcagacgctcgtccgggggcaatgagatatgaaaaagcctgaactcaccgcgacgtatcgggccctggccagctagctagagtcgacctgcaggtccccggggatcggtcttgccttgctcgtcggtgatgtacttcaccagctccgcgaagtcgctcttcttgatggagcgcatggggacgtgcttggcaatcacgcgcaccccccggccgttttagcggctaaaaaagtcatggctctgccctcgggcggaccacgcccatcatgaccttgccaagctcgtcctgcttctcttcgatcttcgccagcagggcgaggatcgtggcatcaccgaaccgcgccgtgcgcgggtcgtcggtgagccagagtttcagcaggccgcccaggcggcccaggtcgccattgatgcgggccagctcgcggacgtgctcatagtccacgacgcccgtgattttgtagccctggccgacggccagcaggtaggccgacaggctcatgccggccgccgccgccttttcctcaatcgctcttcgttcgtctggaaggcagtacaccttgataggtgggctgcccttcctggttggcttggtttcatcagccatccgcttgccctcatctgttacgccggcggtagccggccagcctcgcagagcaggattcccgttgagcaccgccaggtgcgaataagggacagtgaagaaggaacacccgctcgcgggtgggcctacttcacctatcctgcccggctgacgccgttggatacaccaaggaaagtctacacgaaccctttggcaaaatcctgtatatcgtgcgaaaaaggatggatataccgaaaaaatcgctataatgaccccgaagcagggttatgcagcggaaaagatccgtcgacctgcaggcatgc

SEQ ID NO: 15 - DNA, 1185 bp, Unknown
  Vsi-e40pre
atgcgtcgcaccctcaaggccgtgggagcagccgcggcggcggccacctgcgtcctcgccgcgacggcaggcaccgcgcaggccgaggctagcgtctcccacccgttccaccactcctgcgccacggtgaagccgggtcgggcgagctgcaatgccctcgtacgcagcgacatcgcccagagcgcggcgaccctcgcgcaccaagcggccgccccatccgggctctcgccggccaacctgcagagcgcctacaagctgccgtcctccacggccggatccggccagaccgtcgcgatcgtcgacgcctatgacgccccgaccgccgaagcggacttgaacgtgtaccgaagccagttcggactcggcgcgtgcacgaccgccaacggctgtttcaagaaggtcgaccagaacggcggcacgtcctatccgaggaaggacggcggctgggcgcaggagatctccctggacctcgacatggtctccgcggtctgccccaactgcaagatcgttctcgtcgaggcgaagaccaactcgttcgccaacctgggtaccgccgagaacaccgcggcgagtctcgcgaacgtcatcagcaacagctacggcggctcggacgcctctgacgcgagctatggctcgtactacaaccacccgggcaaggccatcacggtcagctccggcgacgccggctacggcgtggagtacccggcctcgtcccactacgtgaccgccgtcggcggcacctcgctgcgcaccgcgagcaccagccgcggctggagcgagaccgcgtggagcggcgcgggcagtggctgctcggcctacaacaccgcgctgtccggccagtccggcctcaccggctgctcccggcgcgccgtcgccgacgtctccgccgtggccgacccggccaccggcgtcgccgtctacgacagcacggcctaccagggccagagcggctggatggtcttcggcggcaccagcgtcgccgcaccgatcatcggtggcgtgtacggcctcgccgccaacgccgcgagcatcgacaacaactacccctacgcccacaccagctcgctcttcgacgtcacgtcgggcagcaacggcacctgcaccaccaccaagtggtgcaccgccggcaccggctgggacggccccaccggcctcggaacgccgaacggcaccggagccttctga

SEQ ID NO: 16 - DNA, 1206 bp, Unknown
  Vsi-e40pre his
atgcgtcgcaccctcaaggccgtgggagcagccgcggcggcggccacctgcgtcctcgccgcgacggcaggcaccgcgcaggccgaggctagcgtctcccacccgttccaccactcctgcgccacggtgaagccgggtcgggcgagctgcaatgccctcgtacgcagcgacatcgcccagagcgcggcgaccctcgcgcaccaagcggccgccccatccgggctctcgccggccaacctgcagagcgcctacaagctgccgtcctccacggccggatccggccagaccgtcgcgatcgtcgacgcctatgacgccccgaccgccgaagcggacttgaacgtgtaccgaagccagttcggactcggcgcgtgcacgaccgccaacggctgtttcaagaaggtcgaccagaacggcggcacgtcctatccgaggaaggacggcggctgggcgcaggagatctccctggacctcgacatggtctccgcggtctgccccaactgcaagatcgttctcgtcgaggcgaagaccaactcgttcgccaacctgggtaccgccgagaacaccgcggcgagtctcgcgaacgtcatcagcaacagctacggcggctcggacgcctctgacgcgagctatggctcgtactacaaccacccgggcaaggccatcacggtcagctccggcgacgccggctacggcgtggagtacccggcctcgtcccactacgtgaccgccgtcggcggcacctcgctgcgcaccgcgagcaccagccgcggctggagcgagaccgcgtggagcggcgcgggcagtggctgctcggcctacaacaccgcgctgtccggccagtccggcctcaccggctgctcccggcgcgccgtcgccgacgtctccgccgtggccgacccggccaccggcgtcgccgtctacgacagcacggcctaccagggccagagcggctggatggtcttcggcggcaccagcgtcgccgcaccgatcatcggtggcgtgtacggcctcgccgccaacgccgcgagcatcgacaacaactacccctacgcccacaccagctcgctcttcgacgtcacgtcgggcagcaacggcacctgcaccaccaccaagtggtgcaccgccggcaccggctgggacggccccaccggcctcggaacgccgaacggcaccggagccttcggacaccaccaccaccaccactga

SEQ ID NO: 17 - DNA, 978 bp, Actinoallomurus
  E40 mat
gccgccccatccgggctctcgccggccaacctgcagagcgcctacaagctgccgtcctccacggccggatccggccagaccgtcgcgatcgtcgacgcctatgacgccccgaccgccgaagcggacttgaacgtgtaccgaagccagttcggactcggcgcgtgcacgaccgccaacggctgtttcaagaaggtcgaccagaacggcggcacgtcctatccgaggaaggacggcggctgggcgcaggagatctccctggacctcgacatggtctccgcggtctgccccaactgcaagatcgttctcgtcgaggcgaagaccaactcgttcgccaacctgggtaccgccgagaacaccgcggcgagtctcgcgaacgtcatcagcaacagctacggcggctcggacgcctctgacgcgagctatggctcgtactacaaccacccgggcaaggccatcacggtcagctccggcgacgccggctacggcgtggagtacccggcctcgtcccactacgtgaccgccgtcggcggcacctcgctgcgcaccgcgagcaccagccgcggctggagcgagaccgcgtggagcggcgcgggcagtggctgctcggcctacaacaccgcgctgtccggccagtccggcctcaccggctgctcccggcgcgccgtcgccgacgtctccgccgtggccgacccggccaccggcgtcgccgtctacgacagcacggcctaccagggccagagcggctggatggtcttcggcggcaccagcgtcgccgcaccgatcatcggtggcgtgtacggcctcgccgccaacgccgcgagcatcgacaacaactacccctacgcccacaccagctcgctcttcgacgtcacgtcgggcagcaacggcacctgcaccaccaccaagtggtgcaccgccggcaccggctgggacggccccaccggcctcggaacgccgaacggcaccggagccttctga

SEQ ID NO: 18 - DNA, 999 bp, Actinoallomurus
  E40 His mat
gccgccccatccgggctctcgccggccaacctgcagagcgcctacaagctgccgtcctccacggccggatccggccagaccgtcgcgatcgtcgacgcctatgacgccccgaccgccgaagcggacttgaacgtgtaccgaagccagttcggactcggcgcgtgcacgaccgccaacggctgtttcaagaaggtcgaccagaacggcggcacgtcctatccgaggaaggacggcggctgggcgcaggagatctccctggacctcgacatggtctccgcggtctgccccaactgcaagatcgttctcgtcgaggcgaagaccaactcgttcgccaacctgggtaccgccgagaacaccgcggcgagtctcgcgaacgtcatcagcaacagctacggcggctcggacgcctctgacgcgagctatggctcgtactacaaccacccgggcaaggccatcacggtcagctccggcgacgccggctacggcgtggagtacccggcctcgtcccactacgtgaccgccgtcggcggcacctcgctgcgcaccgcgagcaccagccgcggctggagcgagaccgcgtggagcggcgcgggcagtggctgctcggcctacaacaccgcgctgtccggccagtccggcctcaccggctgctcccggcgcgccgtcgccgacgtctccgccgtggccgacccggccaccggcgtcgccgtctacgacagcacggcctaccagggccagagcggctggatggtcttcggcggcaccagcgtcgccgcaccgatcatcggtggcgtgtacggcctcgccgccaacgccgcgagcatcgacaacaactacccctacgcccacaccagctcgctcttcgacgtcacgtcgggcagcaacggcacctgcaccaccaccaagtggtgcaccgccggcaccggctgggacggccccaccggcctcggaacgccgaacggcaccggagccttcggacaccaccaccaccaccactga

SEQ ID NO: 19 - DNA, 1811 bp, Unknown
  gusA
atgctgcggcccgtcgaaaccccgacccgcgagatcaagaagctggacggcctgtgggcgttcagcctcgaccgggagaactgcggtatcgaccagcggtggtgggagagcgccctccaggagtcgcgcgccatcgccgtccccggcagcttcaacgaccagttcgcggacgcggacatccgcaactacgcggggaacgtctggtatcagcgggaggtgttcatccccaagggctgggccggtcagcgcatcgtgctgcgcttcgacgccgtgacccactacggcaaggtctgggtcaacaaccaggaagtgatggagcaccagggcggctacacgcccttcgaggcggacgtgaccccgtacgtcatcgccggcaagtcggtccgcatcacggtctgcgtcaacaacgagctcaactggcagaccatcccgcccggcatggtgatcacggacgagaacggcaagaagaagcagagctacttccacgacttcttcaactacgccggcatccaccgctcggtcatgctgtacacgacgccgaacacctgggtcgacgacatcacggtggtcacccacgtggcccaggactgcaaccacgcgtccgtggactggcaggtcgtcgccaacggcgacgtgagcgtggagctccgcgacgccgagcagcaggtcgtggcgaccgggcagggcacctcggggaccctccaggtcgtgaacccccacctctggcagccgggtgagggctacctgtacgagctgtgcgtgacggcgaagagccagaccgagtgcgacatctaccccctgcgcgtcggcatccggtccgtggcggtcaagggcgagcagttcctgatcaaccacaagccgttctacttcacgggcttcggtcggcacgaggacgccgacctccgcggcaagggcttcgacaacgtcctgatggtccacgaccacgccctgatggactggatcggcgccaactcgtaccggacctcgcactacccgtacgcggaagagatgctggactgggcggacgagcacgggatcgtcgtcatcgacgaaaccgccgcggtgggcttcaacctgtccctcggcatcggcttcgaggccggcaacaagccgaaagagctctactccgaagaggccgtcaacggcgaaacccagcaggcccacctccaggcgatcaaagagctcatcgcccgcgacaagaaccacccgtccgtcgtgatgtggtcgatcgccaacgagccggacacccggccgcagggtgcccgggagtacttcgccccgctggccgaggccacccggaagctcgaccccacccggcccatcacctgcgtgaacgtgatgttctgcgacgcccacacggacaccatctccgacctcttcgacgtcctgtgcctgaaccgctactacggctggtacgtgcagtccggggacctggaaacggccgagaaggtcctggagaaagagctgctggcgtggcaggagaagctgcaccagccgatcatcatcaccgagtacggcgtggacacgctggccggtctgcactccatgtacaccgacatgtggtccgaagagtaccagtgcgcgtggctggacatgtaccaccgcgtgttcgaccgcgtcagcgcggtcgtcggcgagcaggtgtggaacttcgccgacttcgccacctcccagggcatcctccgcgtcgggggcaacaagaagggcatcttcacccgggaccgcaagcccaagtcggcggcgttcctgctccagaagcggtggaccgggatgaacttcggggagaagccgcagcagggcgggaagcagtg

SEQ ID NO: 20 - DNA, 1278 bp, Unknown
  kasOp RBS e40 Expression cassette
gtctctgctttgacaacatgctgtgcggtgttgtaaagtctggtgtaggagaatacgacagcttgtcaaaggagtgtccatatgtcacgacgcgtgaccgggaccatactgggcgggttgatcctcgccatggtccccttcctttccaccgcggccaacgccgcaccccaggccgcgccggcttccgtctcccacccgttccaccactcctgcgccacggtgaagccgggtcgggcgagctgcaatgccctcgtacgcagcgacatcgcccagagcgcggcgaccctcgcgcaccaagcggccgccccatccgggctctcgccggccaacctgcagagcgcctacaagctgccgtcctccacggccggatccggccagaccgtcgcgatcgtcgacgcctatgacgccccgaccgccgaagcggacttgaacgtgtaccgaagccagttcggactcggcgcgtgcacgaccgccaacggctgtttcaagaaggtcgaccagaacggcggcacgtcctatccgaggaaggacggcggctgggcgcaggagatctccctggacctcgacatggtctccgcggtctgccccaactgcaagatcgttctcgtcgaggcgaagaccaactcgttcgccaacctgggtaccgccgagaacaccgcggcgagtctcgcgaacgtcatcagcaacagctacggcggctcggacgcctctgacgcgagctatggctcgtactacaaccacccgggcaaggccatcacggtcagctccggcgacgccggctacggcgtggagtacccggcctcgtcccactacgtgaccgccgtcggcggcacctcgctgcgcaccgcgagcaccagccgcggctggagcgagaccgcgtggagcggcgcgggcagtggctgctcggcctacaacaccgcgctgtccggccagtccggcctcaccggctgctcccggcgcgccgtcgccgacgtctccgccgtggccgacccggccaccggcgtcgccgtctacgacagcacggcctaccagggccagagcggctggatggtcttcggcggcaccagcgtcgccgcaccgatcatcggtggcgtgtacggcctcgccgccaacgccgcgagcatcgacaacaactacccctacgcccacaccagctcgctcttcgacgtcacgtcgggcagcaacggcacctgcaccaccaccaagtggtgcaccgccggcaccggctgggacggccccaccggcctcggaacgccgaacggcaccggagccttctga

SEQ ID NO: 21 - DNA, 1299 bp, Unknown
  kasOp RBS e40his Expression cassette
gtctctgctttgacaacatgctgtgcggtgttgtaaagtctggtgtaggagaatacgacagcttgtcaaaggagtgtccatatgtcacgacgcgtgaccgggaccatactgggcgggttgatcctcgccatggtccccttcctttccaccgcggccaacgccgcaccccaggccgcgccggcttccgtctcccacccgttccaccactcctgcgccacggtgaagccgggtcgggcgagctgcaatgccctcgtacgcagcgacatcgcccagagcgcggcgaccctcgcgcaccaagcggccgccccatccgggctctcgccggccaacctgcagagcgcctacaagctgccgtcctccacggccggatccggccagaccgtcgcgatcgtcgacgcctatgacgccccgaccgccgaagcggacttgaacgtgtaccgaagccagttcggactcggcgcgtgcacgaccgccaacggctgtttcaagaaggtcgaccagaacggcggcacgtcctatccgaggaaggacggcggctgggcgcaggagatctccctggacctcgacatggtctccgcggtctgccccaactgcaagatcgttctcgtcgaggcgaagaccaactcgttcgccaacctgggtaccgccgagaacaccgcggcgagtctcgcgaacgtcatcagcaacagctacggcggctcggacgcctctgacgcgagctatggctcgtactacaaccacccgggcaaggccatcacggtcagctccggcgacgccggctacggcgtggagtacccggcctcgtcccactacgtgaccgccgtcggcggcacctcgctgcgcaccgcgagcaccagccgcggctggagcgagaccgcgtggagcggcgcgggcagtggctgctcggcctacaacaccgcgctgtccggccagtccggcctcaccggctgctcccggcgcgccgtcgccgacgtctccgccgtggccgacccggccaccggcgtcgccgtctacgacagcacggcctaccagggccagagcggctggatggtcttcggcggcaccagcgtcgccgcaccgatcatcggtggcgtgtacggcctcgccgccaacgccgcgagcatcgacaacaactacccctacgcccacaccagctcgctcttcgacgtcacgtcgggcagcaacggcacctgcaccaccaccaagtggtgcaccgccggcaccggctgggacggccccaccggcctcggaacgccgaacggcaccggagccttcggacaccaccaccaccaccactga

SEQ ID NO: 22 - DNA, 1266 bp, Unknown
  kasOp RBS vsi-e40 Expression cassette
gtctctgctttgacaacatgctgtgcggtgttgtaaagtctggtgtaggagaatacgacagcttgtcaaaggagtgtccatatgcgtcgcaccctcaaggccgtgggagcagccgcggcggcggccacctgcgtcctcgccgcgacggcaggcaccgcgcaggccgaggctagcgtctcccacccgttccaccactcctgcgccacggtgaagccgggtcgggcgagctgcaatgccctcgtacgcagcgacatcgcccagagcgcggcgaccctcgcgcaccaagcggccgccccatccgggctctcgccggccaacctgcagagcgcctacaagctgccgtcctccacggccggatccggccagaccgtcgcgatcgtcgacgcctatgacgccccgaccgccgaagcggacttgaacgtgtaccgaagccagttcggactcggcgcgtgcacgaccgccaacggctgtttcaagaaggtcgaccagaacggcggcacgtcctatccgaggaaggacggcggctgggcgcaggagatctccctggacctcgacatggtctccgcggtctgccccaactgcaagatcgttctcgtcgaggcgaagaccaactcgttcgccaacctgggtaccgccgagaacaccgcggcgagtctcgcgaacgtcatcagcaacagctacggcggctcggacgcctctgacgcgagctatggctcgtactacaaccacccgggcaaggccatcacggtcagctccggcgacgccggctacggcgtggagtacccggcctcgtcccactacgtgaccgccgtcggcggcacctcgctgcgcaccgcgagcaccagccgcggctggagcgagaccgcgtggagcggcgcgggcagtggctgctcggcctacaacaccgcgctgtccggccagtccggcctcaccggctgctcccggcgcgccgtcgccgacgtctccgccgtggccgacccggccaccggcgtcgccgtctacgacagcacggcctaccagggccagagcggctggatggtcttcggcggcaccagcgtcgccgcaccgatcatcggtggcgtgtacggcctcgccgccaacgccgcgagcatcgacaacaactacccctacgcccacaccagctcgctcttcgacgtcacgtcgggcagcaacggcacctgcaccaccaccaagtggtgcaccgccggcaccggctgggacggccccaccggcctcggaacgccgaacggcaccggagccttctga

SEQ ID NO: 23 - DNA, 1287 bp, Unknown
  kasOp RBS vsi-e40 his Expression cassette
gtctctgctttgacaacatgctgtgcggtgttgtaaagtctggtgtaggagaatacgacagcttgtcaaaggagtgtccatatgcgtcgcaccctcaaggccgtgggagcagccgcggcggcggccacctgcgtcctcgccgcgacggcaggcaccgcgcaggccgaggctagcgtctcccacccgttccaccactcctgcgccacggtgaagccgggtcgggcgagctgcaatgccctcgtacgcagcgacatcgcccagagcgcggcgaccctcgcgcaccaagcggccgccccatccgggctctcgccggccaacctgcagagcgcctacaagctgccgtcctccacggccggatccggccagaccgtcgcgatcgtcgacgcctatgacgccccgaccgccgaagcggacttgaacgtgtaccgaagccagttcggactcggcgcgtgcacgaccgccaacggctgtttcaagaaggtcgaccagaacggcggcacgtcctatccgaggaaggacggcggctgggcgcaggagatctccctggacctcgacatggtctccgcggtctgccccaactgcaagatcgttctcgtcgaggcgaagaccaactcgttcgccaacctgggtaccgccgagaacaccgcggcgagtctcgcgaacgtcatcagcaacagctacggcggctcggacgcctctgacgcgagctatggctcgtactacaaccacccgggcaaggccatcacggtcagctccggcgacgccggctacggcgtggagtacccggcctcgtcccactacgtgaccgccgtcggcggcacctcgctgcgcaccgcgagcaccagccgcggctggagcgagaccgcgtggagcggcgcgggcagtggctgctcggcctacaacaccgcgctgtccggccagtccggcctcaccggctgctcccggcgcgccgtcgccgacgtctccgccgtggccgacccggccaccggcgtcgccgtctacgacagcacggcctaccagggccagagcggctggatggtcttcggcggcaccagcgtcgccgcaccgatcatcggtggcgtgtacggcctcgccgccaacgccgcgagcatcgacaacaactacccctacgcccacaccagctcgctcttcgacgtcacgtcgggcagcaacggcacctgcaccaccaccaagtggtgcaccgccggcaccggctgggacggccccaccggcctcggaacgccgaacggcaccggagccttcggacaccaccaccaccaccactga

SEQ ID NO: 24 - DNA, 1893 bp, Unknown
  kasOp-gusA expression cassette
gtctctgctttgacaacatgctgtgcggtgttgtaaagtctggtgtaggagaatacgacagcttgtcaaaggagtgtccatatgctgcggcccgtcgaaaccccgacccgcgagatcaagaagctggacggcctgtgggcgttcagcctcgaccgggagaactgcggtatcgaccagcggtggtgggagagcgccctccaggagtcgcgcgccatcgccgtccccggcagcttcaacgaccagttcgcggacgcggacatccgcaactacgcggggaacgtctggtatcagcgggaggtgttcatccccaagggctgggccggtcagcgcatcgtgctgcgcttcgacgccgtgacccactacggcaaggtctgggtcaacaaccaggaagtgatggagcaccagggcggctacacgcccttcgaggcggacgtgaccccgtacgtcatcgccggcaagtcggtccgcatcacggtctgcgtcaacaacgagctcaactggcagaccatcccgcccggcatggtgatcacggacgagaacggcaagaagaagcagagctacttccacgacttcttcaactacgccggcatccaccgctcggtcatgctgtacacgacgccgaacacctgggtcgacgacatcacggtggtcacccacgtggcccaggactgcaaccacgcgtccgtggactggcaggtcgtcgccaacggcgacgtgagcgtggagctccgcgacgccgagcagcaggtcgtggcgaccgggcagggcacctcggggaccctccaggtcgtgaacccccacctctggcagccgggtgagggctacctgtacgagctgtgcgtgacggcgaagagccagaccgagtgcgacatctaccccctgcgcgtcggcatccggtccgtggcggtcaagggcgagcagttcctgatcaaccacaagccgttctacttcacgggcttcggtcggcacgaggacgccgacctccgcggcaagggcttcgacaacgtcctgatggtccacgaccacgccctgatggactggatcggcgccaactcgtaccggacctcgcactacccgtacgcggaagagatgctggactgggcggacgagcacgggatcgtcgtcatcgacgaaaccgccgcggtgggcttcaacctgtccctcggcatcggcttcgaggccggcaacaagccgaaagagctctactccgaagaggccgtcaacggcgaaacccagcaggcccacctccaggcgatcaaagagctcatcgcccgcgacaagaaccacccgtccgtcgtgatgtggtcgatcgccaacgagccggacacccggccgcagggtgcccgggagtacttcgccccgctggccgaggccacccggaagctcgaccccacccggcccatcacctgcgtgaacgtgatgttctgcgacgcccacacggacaccatctccgacctcttcgacgtcctgtgcctgaaccgctactacggctggtacgtgcagtccggggacctggaaacggccgagaaggtcctggagaaagagctgctggcgtggcaggagaagctgcaccagccgatcatcatcaccgagtacggcgtggacacgctggccggtctgcactccatgtacaccgacatgtggtccgaagagtaccagtgcgcgtggctggacatgtaccaccgcgtgttcgaccgcgtcagcgcggtcgtcggcgagcaggtgtggaacttcgccgacttcgccacctcccagggcatcctccgcgtcgggggcaacaagaagggcatcttcacccgggaccgcaagcccaagtcggcggcgttcctgctccagaagcggtggaccgggatgaacttcggggagaagccgcagcagggcgggaagcagtga

SEQ ID NO: 25 - DNA, 6913 bp, Unknown
  pMU1s-e40
tggcgccggacggggcttcagacgtttcgggtgctgggttgttgtctctggacagtgatccatgggaaactactcagcaccaccaatgttcccaaaagaaagcgcaggtcagcgcccatgagccaagatctaggcatgtcgcccttcatcgctcccgacgtccctgagcaccttctagacactgttcgcgtcttcctgtacgcgcgtcagtctaagggccggtccgacggctcagacgtgtcgaccgaagcacagctagcggccggtcgtgcgttggtcgcgtctcgcaacgcccaggggggtgcgcgctgggtcgtggcaggtgagttcgtggacgtcgggcgctccggctgggacccgaacgtgacccgtgccgacttcgagcgcatgatgggcgaagtccgcgccggcgaaggtgacgttgtcgttgtgaatgagctttcccggctcactcgcaagggcgcccatgacgcgctcgaaatcgacaacgaattgaagaagcacggcgtgcgcttcatgtcggttcttgagccgttccttgacacgtctacccctatcggcgtcgccattttcgcgctgatcgctgcccttgcgaaacaggacagtgacctgaaggcggagcgcctgaagggtgcgaaagacgagattgccgcgctgggtggcgttcactcgtcttccgccccgttcggaatgcgcgccgtgcgcaagaaggtcgataatctcgtgatctccgttcttgagccggacgaagacaacccggatcacgtcgagctagttgagcgcatggcgaaaatgtcgttcgaaggcgtgtccgacaacgccattgcaacgaccttcgagaaggaaaagatcccgtcgcccggaatggctgagagacgcgccacggaaaagcgtcttgcgtccgtcaaggcacgtcgcctgaacggcgctgaaaagccgatcatgtggcgcgctcaaacggtccgatggattctcaaccatcccgcaatcggcggtttcgcattcgagcgtgtgaagcacggtaaggcgcacatcaacgtcatacggcgcgaccccggcggcaagccgctaacgccccacacgggcattctcagcggctcgaagtggcttgagcttcaagagaagcgttccgggaagaatctcagcgaccggaagcctggggccgaagtcgaaccgacgcttctgagcgggtggcgtttcctggggtgccgaatctgcggcggctcaatgggtcagtcccagggtggccgtaagcgcaacggcgaccttgccgaaggcaattacatgtgcgccaacccgaaggggcacggcggcttgtcggtcaagcgcagcgaactggacgaattcgttgcttcgaaggtgtgggcacggctccgcacagccgacatggaagatgaacacgatcaggcatggattgccgccgctgcggagcgcttcgcccttcagcacgacctagcgggggtggccgatgagcggcgcgaacaacaggcgcacctagacaacgtgcggcgctccatcaaggaccttcaggcggaccgtaagcccggtctgtacgtcgggcgtgaagagctggaaacgtggcgctcaacggtgctgcaataccggtcctacgaagcggagtgcacgacccgactcgctgagcttgacgagaagatgaacggcagcacccgcgttccgtctgagtggttcagcggcgaagacccgacggccgaagggggcatctgggcaagctgggacgtgtacgagcgtcgggagttcctgagcttcttccttgactccgtcatggtcgaccgggggcgccaccctgagacgaagaaatacatccccctgaaggaccgtgtgacgctcaagtgggcggagctgctgaaggaggaagacgaagcgagcgaagccactgagcgggagcttgcggcgctgtagcgcacagcgggaggggtcgagccggcggacggttcggccccttttttggccttgaaatcgttagttaggctaactagggtaccgtctctgctttgacaacatgctgtgcggtgttgtaaagtctggtgtaggagaatacgacagcttgtcaaaggagtgtccatatgtcacgacgcgtgaccgggaccatactgggcgggttgatcctcgccatggtccccttcctttccaccgcggccaacgccgcaccccaggccgcgccggcttccgtctcccacccgttccaccactcctgcgccacggtgaagccgggtcgggcgagctgcaatgccctcgtacgcagcgacatcgcccagagcgcggcgaccctcgcgcaccaagcggccgccccatccgggctctcgccggccaacctgcagagcgcctacaagctgccgtcctccacggccggatccggccagaccgtcgcgatcgtcgacgcctatgacgccccgaccgccgaagcggacttgaacgtgtaccgaagccagttcggactcggcgcgtgcacgaccgccaacggctgtttcaagaaggtcgaccagaacggcggcacgtcctatccgaggaaggacggcggctgggcgcaggagatctccctggacctcgacatggtctccgcggtctgccccaactgcaagatcgttctcgtcgaggcgaagaccaactcgttcgccaacctgggtaccgccgagaacaccgcggcgagtctcgcgaacgtcatcagcaacagctacggcggctcggacgcctctgacgcgagctatggctcgtactacaaccacccgggcaaggccatcacggtcagctccggcgacgccggctacggcgtggagtacccggcctcgtcccactacgtgaccgccgtcggcggcacctcgctgcgcaccgcgagcaccagccgcggctggagcgagaccgcgtggagcggcgcgggcagtggctgctcggcctacaacaccgcgctgtccggccagtccggcctcaccggctgctcccggcgcgccgtcgccgacgtctccgccgtggccgacccggccaccggcgtcgccgtctacgacagcacggcctaccagggccagagcggctggatggtcttcggcggcaccagcgtcgccgcaccgatcatcggtggcgtgtacggcctcgccgccaacgccgcgagcatcgacaacaactacccctacgcccacaccagctcgctcttcgacgtcacgtcgggcagcaacggcacctgcaccaccaccaagtggtgcaccgccggcaccggctgggacggccccaccggcctcggaacgccgaacggcaccggagccttctgaagcttactaggtatctagaaccggtgacgtcaccatgggaagcttcgtggatccagatatccctctagaccgcggccgcccggctgcagcccgtacctctagtagagtcgagggggaacccggccgcgtccggcgcccccgccgccttcgacgagatcccgcaaaagcggcctttgactccctgcaagcctcagcgaccgaatatatcggttatgcgtgggcgatggttgttgtcattgtcggcgcaactatcggtatcaagctgtttaagaaattcacctcgaaagcaagctgataaaccgatacaattaaaggctccttttggagcctttttttttggagattttcaacgtgaaaaaattattattcgcaattcctttagttgttcctttctattctcactccgctgaaactgttgaaagttgtttagcaaaacctcatacagaaaattcatttactaacgtctggaaagacgacaaaactttagatcctctagctagagtcgaccggcatgcaatcgaattcgtaatcatgtcatagctgtttcctgtgtgaaattgttatccgctcacaattccacacaacatacgagccggaagcataaagtgtaaagcctggggtgcctaatgagtgagctaactcacattaattgcgttgcgctcactgcccgctttccagtcgggaaacctgtcgtgccagctgcattaatgaatcggccaacgcgcggggagaggcggtttgcgtattgggcgctcttccgcttcctcgctcactgactcgctgcgctcggtcgttcggctgcggcgagcggtatcagctcactcaaaggcggtaatacggttatccacagaatcaggggataacgcaggaaagaacatgtgagcaaaaggccagcaaaaggccaggaaccgtaaaaaggccgcgttgctggcgtttttccataggctccgcccccctgacgagcatcacaaaaatcgacgctcaagtcagaggtggcgaaacccgacaggactataaagataccaggcgtttccccctggaagctccctcgtgcgctctcctgttccgaccctgccgcttaccggatacctgtccgcctttctcccttcgggaagcgtggcgctttctcatagctcacgctgtaggtatctcagttcggtgtaggtcgttcgctccaagctgggctgtgtgcacgaaccccccgttcagcccgaccgctgcgccttatccggtaactatcgtcttgagtccaacccggtaagacacgacttatcgccactggcagcagccactggtaacaggattagcagagcgaggtatgtaggcggtgctacagagttcttgaagtggtggcctaactacggctacactagaagaacagtatttggtatctgcgctctgctgaagccagttaccttcggaaaaagagttggtagctcttgatccggcaaacaaaccaccgctggtagcggtggtttttttgtttgcaagcagcagattacgcgcagaaaaaaaggatctcaagaagatcctttgatcttttctacggggtctgacgctcagtggaacgaaaactcacgttaagggattttggtcatgagattatcaaaaaggatcttcacctagatccttttggttcatgtgcagctccatcagcaaaaggggatgataagtttatcaccaccgactatttgcaacagtgccgttgatcgtgctatgatcgactgatgtcatcagcggtggagtgcaatgtcgtgcaatacgaatggcgaaaagccgagctcatcggtcagcttctcaaccttggggttacccccggcggtgtgctgctggtccacagctccttccgtagcgtccggcccctcgaagatgggccacttggactgatcgaggccctgcgtgctgcgctgggtccgggagggacgctcgtcatgccctcgtggtcaggtctggacgacgagccgttcgatcctgccacgtcgcccgttacaccggaccttggagttgtctctgacacattctggcgcctgccaaatgtaaagcgcagcgcccatccatttgcctttgcggcagcggggccacaggcagagcagatcatctctgatccattgcccctgccacctcactcgcctgcaagcccggtcgcccgtgtccatgaactcgatgggcaggtacttctcctcggcgtgggacacgatgccaacacgacgctgcatcttgccgagttgatggcaaaggttccctatggggtgccgagacactgcaccattcttcaggatggcaagttggtacgcgtcgattatctcgagaatgaccactgctgtgagcgctttgccttggcggacaggtggctcaaggagaagagccttcagaaggaaggtccagtcggtcatgcctttgctcggttgatccgctcccgcgacattgtggcgacagccctgggtcaactgggccgagatccgttgatcttcctgcatccgccagaggcgggatgcgaagaatgcgatgccgctcgccagtcgattggctgagctcatgagcggagaacgagatgacgttggaggggcaaggtcgcgctgattgctggggcaacacgtggagcggatcggggattgtctttcttcagctcgctgatgatatgctgacgctcaatgccgtttggcctccgactaacgaaaatcccgcatttggacggctgatccgattggcacggcggacggcgaatggcggagcagacgctcgtccgggggcaatgagatatgaaaaagcctgaactcaccgcgacgtatcgggccctggccagctagctagagtcgacctgcaggtccccggggatcggtcttgccttgctcgtcggtgatgtacttcaccagctccgcgaagtcgctcttcttgatggagcgcatggggacgtgcttggcaatcacgcgcaccccccggccgttttagcggctaaaaaagtcatggctctgccctcgggcggaccacgcccatcatgaccttgccaagctcgtcctgcttctcttcgatcttcgccagcagggcgaggatcgtggcatcaccgaaccgcgccgtgcgcgggtcgtcggtgagccagagtttcagcaggccgcccaggcggcccaggtcgccattgatgcgggccagctcgcggacgtgctcatagtccacgacgcccgtgattttgtagccctggccgacggccagcaggtaggccgacaggctcatgccggccgccgccgccttttcctcaatcgctcttcgttcgtctggaaggcagtacaccttgataggtgggctgcccttcctggttggcttggtttcatcagccatccgcttgccctcatctgttacgccggcggtagccggccagcctcgcagagcaggattcccgttgagcaccgccaggtgcgaataagggacagtgaagaaggaacacccgctcgcgggtgggcctacttcacctatcctgcccggctgacgccgttggatacaccaaggaaagtctacacgaaccctttggcaaaatcctgtatatcgtgcgaaaaaggatggatataccgaaaaaatcgctataatgaccccgaagcagggttatgcagcggaaaagatccgtcgacctgcaggcatgc

SEQ ID NO: 26 - DNA, 6934 bp, Unknown
  pMU1s-e40His
tggcgccggacggggcttcagacgtttcgggtgctgggttgttgtctctggacagtgatccatgggaaactactcagcaccaccaatgttcccaaaagaaagcgcaggtcagcgcccatgagccaagatctaggcatgtcgcccttcatcgctcccgacgtccctgagcaccttctagacactgttcgcgtcttcctgtacgcgcgtcagtctaagggccggtccgacggctcagacgtgtcgaccgaagcacagctagcggccggtcgtgcgttggtcgcgtctcgcaacgcccaggggggtgcgcgctgggtcgtggcaggtgagttcgtggacgtcgggcgctccggctgggacccgaacgtgacccgtgccgacttcgagcgcatgatgggcgaagtccgcgccggcgaaggtgacgttgtcgttgtgaatgagctttcccggctcactcgcaagggcgcccatgacgcgctcgaaatcgacaacgaattgaagaagcacggcgtgcgcttcatgtcggttcttgagccgttccttgacacgtctacccctatcggcgtcgccattttcgcgctgatcgctgcccttgcgaaacaggacagtgacctgaaggcggagcgcctgaagggtgcgaaagacgagattgccgcgctgggtggcgttcactcgtcttccgccccgttcggaatgcgcgccgtgcgcaagaaggtcgataatctcgtgatctccgttcttgagccggacgaagacaacccggatcacgtcgagctagttgagcgcatggcgaaaatgtcgttcgaaggcgtgtccgacaacgccattgcaacgaccttcgagaaggaaaagatcccgtcgcccggaatggctgagagacgcgccacggaaaagcgtcttgcgtccgtcaaggcacgtcgcctgaacggcgctgaaaagccgatcatgtggcgcgctcaaacggtccgatggattctcaaccatcccgcaatcggcggtttcgcattcgagcgtgtgaagcacggtaaggcgcacatcaacgtcatacggcgcgaccccggcggcaagccgctaacgccccacacgggcattctcagcggctcgaagtggcttgagcttcaagagaagcgttccgggaagaatctcagcgaccggaagcctggggccgaagtcgaaccgacgcttctgagcgggtggcgtttcctggggtgccgaatctgcggcggctcaatgggtcagtcccagggtggccgtaagcgcaacggcgaccttgccgaaggcaattacatgtgcgccaacccgaaggggcacggcggcttgtcggtcaagcgcagcgaactggacgaattcgttgcttcgaaggtgtgggcacggctccgcacagccgacatggaagatgaacacgatcaggcatggattgccgccgctgcggagcgcttcgcccttcagcacgacctagcgggggtggccgatgagcggcgcgaacaacaggcgcacctagacaacgtgcggcgctccatcaaggaccttcaggcggaccgtaagcccggtctgtacgtcgggcgtgaagagctggaaacgtggcgctcaacggtgctgcaataccggtcctacgaagcggagtgcacgacccgactcgctgagcttgacgagaagatgaacggcagcacccgcgttccgtctgagtggttcagcggcgaagacccgacggccgaagggggcatctgggcaagctgggacgtgtacgagcgtcgggagttcctgagcttcttccttgactccgtcatggtcgaccgggggcgccaccctgagacgaagaaatacatccccctgaaggaccgtgtgacgctcaagtgggcggagctgctgaaggaggaagacgaagcgagcgaagccactgagcgggagcttgcggcgctgtagcgcacagcgggaggggtcgagccggcggacggttcggccccttttttggccttgaaatcgttagttaggctaactagggtaccgtctctgctttgacaacatgctgtgcggtgttgtaaagtctggtgtaggagaatacgacagcttgtcaaaggagtgtccatatgtcacgacgcgtgaccgggaccatactgggcgggttgatcctcgccatggtccccttcctttccaccgcggccaacgccgcaccccaggccgcgccggcttccgtctcccacccgttccaccactcctgcgccacggtgaagccgggtcgggcgagctgcaatgccctcgtacgcagcgacatcgcccagagcgcggcgaccctcgcgcaccaagcggccgccccatccgggctctcgccggccaacctgcagagcgcctacaagctgccgtcctccacggccggatccggccagaccgtcgcgatcgtcgacgcctatgacgccccgaccgccgaagcggacttgaacgtgtaccgaagccagttcggactcggcgcgtgcacgaccgccaacggctgtttcaagaaggtcgaccagaacggcggcacgtcctatccgaggaaggacggcggctgggcgcaggagatctccctggacctcgacatggtctccgcggtctgccccaactgcaagatcgttctcgtcgaggcgaagaccaactcgttcgccaacctgggtaccgccgagaacaccgcggcgagtctcgcgaacgtcatcagcaacagctacggcggctcggacgcctctgacgcgagctatggctcgtactacaaccacccgggcaaggccatcacggtcagctccggcgacgccggctacggcgtggagtacccggcctcgtcccactacgtgaccgccgtcggcggcacctcgctgcgcaccgcgagcaccagccgcggctggagcgagaccgcgtggagcggcgcgggcagtggctgctcggcctacaacaccgcgctgtccggccagtccggcctcaccggctgctcccggcgcgccgtcgccgacgtctccgccgtggccgacccggccaccggcgtcgccgtctacgacagcacggcctaccagggccagagcggctggatggtcttcggcggcaccagcgtcgccgcaccgatcatcggtggcgtgtacggcctcgccgccaacgccgcgagcatcgacaacaactacccctacgcccacaccagctcgctcttcgacgtcacgtcgggcagcaacggcacctgcaccaccaccaagtggtgcaccgccggcaccggctgggacggccccaccggcctcggaacgccgaacggcaccggagccttcggacaccaccaccaccaccactgaagcttactaggtatctagaaccggtgacgtcaccatgggaagcttcgtggatccagatatccctctagaccgcggccgcccggctgcagcccgtacctctagtagagtcgagggggaacccggccgcgtccggcgcccccgccgccttcgacgagatcccgcaaaagcggcctttgactccctgcaagcctcagcgaccgaatatatcggttatgcgtgggcgatggttgttgtcattgtcggcgcaactatcggtatcaagctgtttaagaaattcacctcgaaagcaagctgataaaccgatacaattaaaggctccttttggagcctttttttttggagattttcaacgtgaaaaaattattattcgcaattcctttagttgttcctttctattctcactccgctgaaactgttgaaagttgtttagcaaaacctcatacagaaaattcatttactaacgtctggaaagacgacaaaactttagatcctctagctagagtcgaccggcatgcaatcgaattcgtaatcatgtcatagctgtttcctgtgtgaaattgttatccgctcacaattccacacaacatacgagccggaagcataaagtgtaaagcctggggtgcctaatgagtgagctaactcacattaattgcgttgcgctcactgcccgctttccagtcgggaaacctgtcgtgccagctgcattaatgaatcggccaacgcgcggggagaggcggtttgcgtattgggcgctcttccgcttcctcgctcactgactcgctgcgctcggtcgttcggctgcggcgagcggtatcagctcactcaaaggcggtaatacggttatccacagaatcaggggataacgcaggaaagaacatgtgagcaaaaggccagcaaaaggccaggaaccgtaaaaaggccgcgttgctggcgtttttccataggctccgcccccctgacgagcatcacaaaaatcgacgctcaagtcagaggtggcgaaacccgacaggactataaagataccaggcgtttccccctggaagctccctcgtgcgctctcctgttccgaccctgccgcttaccggatacctgtccgcctttctcccttcgggaagcgtggcgctttctcatagctcacgctgtaggtatctcagttcggtgtaggtcgttcgctccaagctgggctgtgtgcacgaaccccccgttcagcccgaccgctgcgccttatccggtaactatcgtcttgagtccaacccggtaagacacgacttatcgccactggcagcagccactggtaacaggattagcagagcgaggtatgtaggcggtgctacagagttcttgaagtggtggcctaactacggctacactagaagaacagtatttggtatctgcgctctgctgaagccagttaccttcggaaaaagagttggtagctcttgatccggcaaacaaaccaccgctggtagcggtggtttttttgtttgcaagcagcagattacgcgcagaaaaaaaggatctcaagaagatcctttgatcttttctacggggtctgacgctcagtggaacgaaaactcacgttaagggattttggtcatgagattatcaaaaaggatcttcacctagatccttttggttcatgtgcagctccatcagcaaaaggggatgataagtttatcaccaccgactatttgcaacagtgccgttgatcgtgctatgatcgactgatgtcatcagcggtggagtgcaatgtcgtgcaatacgaatggcgaaaagccgagctcatcggtcagcttctcaaccttggggttacccccggcggtgtgctgctggtccacagctccttccgtagcgtccggcccctcgaagatgggccacttggactgatcgaggccctgcgtgctgcgctgggtccgggagggacgctcgtcatgccctcgtggtcaggtctggacgacgagccgttcgatcctgccacgtcgcccgttacaccggaccttggagttgtctctgacacattctggcgcctgccaaatgtaaagcgcagcgcccatccatttgcctttgcggcagcggggccacaggcagagcagatcatctctgatccattgcccctgccacctcactcgcctgcaagcccggtcgcccgtgtccatgaactcgatgggcaggtacttctcctcggcgtgggacacgatgccaacacgacgctgcatcttgccgagttgatggcaaaggttccctatggggtgccgagacactgcaccattcttcaggatggcaagttggtacgcgtcgattatctcgagaatgaccactgctgtgagcgctttgccttggcggacaggtggctcaaggagaagagccttcagaaggaaggtccagtcggtcatgcctttgctcggttgatccgctcccgcgacattgtggcgacagccctgggtcaactgggccgagatccgttgatcttcctgcatccgccagaggcgggatgcgaagaatgcgatgccgctcgccagtcgattggctgagctcatgagcggagaacgagatgacgttggaggggcaaggtcgcgctgattgctggggcaacacgtggagcggatcggggattgtctttcttcagctcgctgatgatatgctgacgctcaatgccgtttggcctccgactaacgaaaatcccgcatttggacggctgatccgattggcacggcggacggcgaatggcggagcagacgctcgtccgggggcaatgagatatgaaaaagcctgaactcaccgcgacgtatcgggccctggccagctagctagagtcgacctgcaggtccccggggatcggtcttgccttgctcgtcggtgatgtacttcaccagctccgcgaagtcgctcttcttgatggagcgcatggggacgtgcttggcaatcacgcgcaccccccggccgttttagcggctaaaaaagtcatggctctgccctcgggcggaccacgcccatcatgaccttgccaagctcgtcctgcttctcttcgatcttcgccagcagggcgaggatcgtggcatcaccgaaccgcgccgtgcgcgggtcgtcggtgagccagagtttcagcaggccgcccaggcggcccaggtcgccattgatgcgggccagctcgcggacgtgctcatagtccacgacgcccgtgattttgtagccctggccgacggccagcaggtaggccgacaggctcatgccggccgccgccgccttttcctcaatcgctcttcgttcgtctggaaggcagtacaccttgataggtgggctgcccttcctggttggcttggtttcatcagccatccgcttgccctcatctgttacgccggcggtagccggccagcctcgcagagcaggattcccgttgagcaccgccaggtgcgaataagggacagtgaagaaggaacacccgctcgcgggtgggcctacttcacctatcctgcccggctgacgccgttggatacaccaaggaaagtctacacgaaccctttggcaaaatcctgtatatcgtgcgaaaaaggatggatataccgaaaaaatcgctataatgaccccgaagcagggttatgcagcggaaaagatccgtcgacctgcaggcatgc

SEQ ID NO: 27 - DNA, 6901 bp, Unknown
  pMU1s-vsie40pre
tggcgccggacggggcttcagacgtttcgggtgctgggttgttgtctctggacagtgatccatgggaaactactcagcaccaccaatgttcccaaaagaaagcgcaggtcagcgcccatgagccaagatctaggcatgtcgcccttcatcgctcccgacgtccctgagcaccttctagacactgttcgcgtcttcctgtacgcgcgtcagtctaagggccggtccgacggctcagacgtgtcgaccgaagcacagctagcggccggtcgtgcgttggtcgcgtctcgcaacgcccaggggggtgcgcgctgggtcgtggcaggtgagttcgtggacgtcgggcgctccggctgggacccgaacgtgacccgtgccgacttcgagcgcatgatgggcgaagtccgcgccggcgaaggtgacgttgtcgttgtgaatgagctttcccggctcactcgcaagggcgcccatgacgcgctcgaaatcgacaacgaattgaagaagcacggcgtgcgcttcatgtcggttcttgagccgttccttgacacgtctacccctatcggcgtcgccattttcgcgctgatcgctgcccttgcgaaacaggacagtgacctgaaggcggagcgcctgaagggtgcgaaagacgagattgccgcgctgggtggcgttcactcgtcttccgccccgttcggaatgcgcgccgtgcgcaagaaggtcgataatctcgtgatctccgttcttgagccggacgaagacaacccggatcacgtcgagctagttgagcgcatggcgaaaatgtcgttcgaaggcgtgtccgacaacgccattgcaacgaccttcgagaaggaaaagatcccgtcgcccggaatggctgagagacgcgccacggaaaagcgtcttgcgtccgtcaaggcacgtcgcctgaacggcgctgaaaagccgatcatgtggcgcgctcaaacggtccgatggattctcaaccatcccgcaatcggcggtttcgcattcgagcgtgtgaagcacggtaaggcgcacatcaacgtcatacggcgcgaccccggcggcaagccgctaacgccccacacgggcattctcagcggctcgaagtggcttgagcttcaagagaagcgttccgggaagaatctcagcgaccggaagcctggggccgaagtcgaaccgacgcttctgagcgggtggcgtttcctggggtgccgaatctgcggcggctcaatgggtcagtcccagggtggccgtaagcgcaacggcgaccttgccgaaggcaattacatgtgcgccaacccgaaggggcacggcggcttgtcggtcaagcgcagcgaactggacgaattcgttgcttcgaaggtgtgggcacggctccgcacagccgacatggaagatgaacacgatcaggcatggattgccgccgctgcggagcgcttcgcccttcagcacgacctagcgggggtggccgatgagcggcgcgaacaacaggcgcacctagacaacgtgcggcgctccatcaaggaccttcaggcggaccgtaagcccggtctgtacgtcgggcgtgaagagctggaaacgtggcgctcaacggtgctgcaataccggtcctacgaagcggagtgcacgacccgactcgctgagcttgacgagaagatgaacggcagcacccgcgttccgtctgagtggttcagcggcgaagacccgacggccgaagggggcatctgggcaagctgggacgtgtacgagcgtcgggagttcctgagcttcttccttgactccgtcatggtcgaccgggggcgccaccctgagacgaagaaatacatccccctgaaggaccgtgtgacgctcaagtgggcggagctgctgaaggaggaagacgaagcgagcgaagccactgagcgggagcttgcggcgctgtagcgcacagcgggaggggtcgagccggcggacggttcggccccttttttggccttgaaatcgttagttaggctaactagggtaccgtctctgctttgacaacatgctgtgcggtgttgtaaagtctggtgtaggagaatacgacagcttgtcaaaggagtgtccatatgcgtcgcaccctcaaggccgtgggagcagccgcggcggcggccacctgcgtcctcgccgcgacggcaggcaccgcgcaggccgaggctagcgtctcccacccgttccaccactcctgcgccacggtgaagccgggtcgggcgagctgcaatgccctcgtacgcagcgacatcgcccagagcgcggcgaccctcgcgcaccaagcggccgccccatccgggctctcgccggccaacctgcagagcgcctacaagctgccgtcctccacggccggatccggccagaccgtcgcgatcgtcgacgcctatgacgccccgaccgccgaagcggacttgaacgtgtaccgaagccagttcggactcggcgcgtgcacgaccgccaacggctgtttcaagaaggtcgaccagaacggcggcacgtcctatccgaggaaggacggcggctgggcgcaggagatctccctggacctcgacatggtctccgcggtctgccccaactgcaagatcgttctcgtcgaggcgaagaccaactcgttcgccaacctgggtaccgccgagaacaccgcggcgagtctcgcgaacgtcatcagcaacagctacggcggctcggacgcctctgacgcgagctatggctcgtactacaaccacccgggcaaggccatcacggtcagctccggcgacgccggctacggcgtggagtacccggcctcgtcccactacgtgaccgccgtcggcggcacctcgctgcgcaccgcgagcaccagccgcggctggagcgagaccgcgtggagcggcgcgggcagtggctgctcggcctacaacaccgcgctgtccggccagtccggcctcaccggctgctcccggcgcgccgtcgccgacgtctccgccgtggccgacccggccaccggcgtcgccgtctacgacagcacggcctaccagggccagagcggctggatggtcttcggcggcaccagcgtcgccgcaccgatcatcggtggcgtgtacggcctcgccgccaacgccgcgagcatcgacaacaactacccctacgcccacaccagctcgctcttcgacgtcacgtcgggcagcaacggcacctgcaccaccaccaagtggtgcaccgccggcaccggctgggacggccccaccggcctcggaacgccgaacggcaccggagccttctgaagcttactaggtatctagaaccggtgacgtcaccatgggaagcttcgtggatccagatatccctctagaccgcggccgcccggctgcagcccgtacctctagtagagtcgagggggaacccggccgcgtccggcgcccccgccgccttcgacgagatcccgcaaaagcggcctttgactccctgcaagcctcagcgaccgaatatatcggttatgcgtgggcgatggttgttgtcattgtcggcgcaactatcggtatcaagctgtttaagaaattcacctcgaaagcaagctgataaaccgatacaattaaaggctccttttggagcctttttttttggagattttcaacgtgaaaaaattattattcgcaattcctttagttgttcctttctattctcactccgctgaaactgttgaaagttgtttagcaaaacctcatacagaaaattcatttactaacgtctggaaagacgacaaaactttagatcctctagctagagtcgaccggcatgcaatcgaattcgtaatcatgtcatagctgtttcctgtgtgaaattgttatccgctcacaattccacacaacatacgagccggaagcataaagtgtaaagcctggggtgcctaatgagtgagctaactcacattaattgcgttgcgctcactgcccgctttccagtcgggaaacctgtcgtgccagctgcattaatgaatcggccaacgcgcggggagaggcggtttgcgtattgggcgctcttccgcttcctcgctcactgactcgctgcgctcggtcgttcggctgcggcgagcggtatcagctcactcaaaggcggtaatacggttatccacagaatcaggggataacgcaggaaagaacatgtgagcaaaaggccagcaaaaggccaggaaccgtaaaaaggccgcgttgctggcgtttttccataggctccgcccccctgacgagcatcacaaaaatcgacgctcaagtcagaggtggcgaaacccgacaggactataaagataccaggcgtttccccctggaagctccctcgtgcgctctcctgttccgaccctgccgcttaccggatacctgtccgcctttctcccttcgggaagcgtggcgctttctcatagctcacgctgtaggtatctcagttcggtgtaggtcgttcgctccaagctgggctgtgtgcacgaaccccccgttcagcccgaccgctgcgccttatccggtaactatcgtcttgagtccaacccggtaagacacgacttatcgccactggcagcagccactggtaacaggattagcagagcgaggtatgtaggcggtgctacagagttcttgaagtggtggcctaactacggctacactagaagaacagtatttggtatctgcgctctgctgaagccagttaccttcggaaaaagagttggtagctcttgatccggcaaacaaaccaccgctggtagcggtggtttttttgtttgcaagcagcagattacgcgcagaaaaaaaggatctcaagaagatcctttgatcttttctacggggtctgacgctcagtggaacgaaaactcacgttaagggattttggtcatgagattatcaaaaaggatcttcacctagatccttttggttcatgtgcagctccatcagcaaaaggggatgataagtttatcaccaccgactatttgcaacagtgccgttgatcgtgctatgatcgactgatgtcatcagcggtggagtgcaatgtcgtgcaatacgaatggcgaaaagccgagctcatcggtcagcttctcaaccttggggttacccccggcggtgtgctgctggtccacagctccttccgtagcgtccggcccctcgaagatgggccacttggactgatcgaggccctgcgtgctgcgctgggtccgggagggacgctcgtcatgccctcgtggtcaggtctggacgacgagccgttcgatcctgccacgtcgcccgttacaccggaccttggagttgtctctgacacattctggcgcctgccaaatgtaaagcgcagcgcccatccatttgcctttgcggcagcggggccacaggcagagcagatcatctctgatccattgcccctgccacctcactcgcctgcaagcccggtcgcccgtgtccatgaactcgatgggcaggtacttctcctcggcgtgggacacgatgccaacacgacgctgcatcttgccgagttgatggcaaaggttccctatggggtgccgagacactgcaccattcttcaggatggcaagttggtacgcgtcgattatctcgagaatgaccactgctgtgagcgctttgccttggcggacaggtggctcaaggagaagagccttcagaaggaaggtccagtcggtcatgcctttgctcggttgatccgctcccgcgacattgtggcgacagccctgggtcaactgggccgagatccgttgatcttcctgcatccgccagaggcgggatgcgaagaatgcgatgccgctcgccagtcgattggctgagctcatgagcggagaacgagatgacgttggaggggcaaggtcgcgctgattgctggggcaacacgtggagcggatcggggattgtctttcttcagctcgctgatgatatgctgacgctcaatgccgtttggcctccgactaacgaaaatcccgcatttggacggctgatccgattggcacggcggacggcgaatggcggagcagacgctcgtccgggggcaatgagatatgaaaaagcctgaactcaccgcgacgtatcgggccctggccagctagctagagtcgacctgcaggtccccggggatcggtcttgccttgctcgtcggtgatgtacttcaccagctccgcgaagtcgctcttcttgatggagcgcatggggacgtgcttggcaatcacgcgcaccccccggccgttttagcggctaaaaaagtcatggctctgccctcgggcggaccacgcccatcatgaccttgccaagctcgtcctgcttctcttcgatcttcgccagcagggcgaggatcgtggcatcaccgaaccgcgccgtgcgcgggtcgtcggtgagccagagtttcagcaggccgcccaggcggcccaggtcgccattgatgcgggccagctcgcggacgtgctcatagtccacgacgcccgtgattttgtagccctggccgacggccagcaggtaggccgacaggctcatgccggccgccgccgccttttcctcaatcgctcttcgttcgtctggaaggcagtacaccttgataggtgggctgcccttcctggttggcttggtttcatcagccatccgcttgccctcatctgttacgccggcggtagccggccagcctcgcagagcaggattcccgttgagcaccgccaggtgcgaataagggacagtgaagaaggaacacccgctcgcgggtgggcctacttcacctatcctgcccggctgacgccgttggatacaccaaggaaagtctacacgaaccctttggcaaaatcctgtatatcgtgcgaaaaaggatggatataccgaaaaaatcgctataatgaccccgaagcagggttatgcagcggaaaagatccgtcgacctgcaggcatgc

SEQ ID NO: 28 - DNA, 6922 bp, Unknown
  pMU1s-vsie40Hispre
tggcgccggacggggcttcagacgtttcgggtgctgggttgttgtctctggacagtgatccatgggaaactactcagcaccaccaatgttcccaaaagaaagcgcaggtcagcgcccatgagccaagatctaggcatgtcgcccttcatcgctcccgacgtccctgagcaccttctagacactgttcgcgtcttcctgtacgcgcgtcagtctaagggccggtccgacggctcagacgtgtcgaccgaagcacagctagcggccggtcgtgcgttggtcgcgtctcgcaacgcccaggggggtgcgcgctgggtcgtggcaggtgagttcgtggacgtcgggcgctccggctgggacccgaacgtgacccgtgccgacttcgagcgcatgatgggcgaagtccgcgccggcgaaggtgacgttgtcgttgtgaatgagctttcccggctcactcgcaagggcgcccatgacgcgctcgaaatcgacaacgaattgaagaagcacggcgtgcgcttcatgtcggttcttgagccgttccttgacacgtctacccctatcggcgtcgccattttcgcgctgatcgctgcccttgcgaaacaggacagtgacctgaaggcggagcgcctgaagggtgcgaaagacgagattgccgcgctgggtggcgttcactcgtcttccgccccgttcggaatgcgcgccgtgcgcaagaaggtcgataatctcgtgatctccgttcttgagccggacgaagacaacccggatcacgtcgagctagttgagcgcatggcgaaaatgtcgttcgaaggcgtgtccgacaacgccattgcaacgaccttcgagaaggaaaagatcccgtcgcccggaatggctgagagacgcgccacggaaaagcgtcttgcgtccgtcaaggcacgtcgcctgaacggcgctgaaaagccgatcatgtggcgcgctcaaacggtccgatggattctcaaccatcccgcaatcggcggtttcgcattcgagcgtgtgaagcacggtaaggcgcacatcaacgtcatacggcgcgaccccggcggcaagccgctaacgccccacacgggcattctcagcggctcgaagtggcttgagcttcaagagaagcgttccgggaagaatctcagcgaccggaagcctggggccgaagtcgaaccgacgcttctgagcgggtggcgtttcctggggtgccgaatctgcggcggctcaatgggtcagtcccagggtggccgtaagcgcaacggcgaccttgccgaaggcaattacatgtgcgccaacccgaaggggcacggcggcttgtcggtcaagcgcagcgaactggacgaattcgttgcttcgaaggtgtgggcacggctccgcacagccgacatggaagatgaacacgatcaggcatggattgccgccgctgcggagcgcttcgcccttcagcacgacctagcgggggtggccgatgagcggcgcgaacaacaggcgcacctagacaacgtgcggcgctccatcaaggaccttcaggcggaccgtaagcccggtctgtacgtcgggcgtgaagagctggaaacgtggcgctcaacggtgctgcaataccggtcctacgaagcggagtgcacgacccgactcgctgagcttgacgagaagatgaacggcagcacccgcgttccgtctgagtggttcagcggcgaagacccgacggccgaagggggcatctgggcaagctgggacgtgtacgagcgtcgggagttcctgagcttcttccttgactccgtcatggtcgaccgggggcgccaccctgagacgaagaaatacatccccctgaaggaccgtgtgacgctcaagtgggcggagctgctgaaggaggaagacgaagcgagcgaagccactgagcgggagcttgcggcgctgtagcgcacagcgggaggggtcgagccggcggacggttcggccccttttttggccttgaaatcgttagttaggctaactagggtaccgtctctgctttgacaacatgctgtgcggtgttgtaaagtctggtgtaggagaatacgacagcttgtcaaaggagtgtccatatgcgtcgcaccctcaaggccgtgggagcagccgcggcggcggccacctgcgtcctcgccgcgacggcaggcaccgcgcaggccgaggctagcgtctcccacccgttccaccactcctgcgccacggtgaagccgggtcgggcgagctgcaatgccctcgtacgcagcgacatcgcccagagcgcggcgaccctcgcgcaccaagcggccgccccatccgggctctcgccggccaacctgcagagcgcctacaagctgccgtcctccacggccggatccggccagaccgtcgcgatcgtcgacgcctatgacgccccgaccgccgaagcggacttgaacgtgtaccgaagccagttcggactcggcgcgtgcacgaccgccaacggctgtttcaagaaggtcgaccagaacggcggcacgtcctatccgaggaaggacggcggctgggcgcaggagatctccctggacctcgacatggtctccgcggtctgccccaactgcaagatcgttctcgtcgaggcgaagaccaactcgttcgccaacctgggtaccgccgagaacaccgcggcgagtctcgcgaacgtcatcagcaacagctacggcggctcggacgcctctgacgcgagctatggctcgtactacaaccacccgggcaaggccatcacggtcagctccggcgacgccggctacggcgtggagtacccggcctcgtcccactacgtgaccgccgtcggcggcacctcgctgcgcaccgcgagcaccagccgcggctggagcgagaccgcgtggagcggcgcgggcagtggctgctcggcctacaacaccgcgctgtccggccagtccggcctcaccggctgctcccggcgcgccgtcgccgacgtctccgccgtggccgacccggccaccggcgtcgccgtctacgacagcacggcctaccagggccagagcggctggatggtcttcggcggcaccagcgtcgccgcaccgatcatcggtggcgtgtacggcctcgccgccaacgccgcgagcatcgacaacaactacccctacgcccacaccagctcgctcttcgacgtcacgtcgggcagcaacggcacctgcaccaccaccaagtggtgcaccgccggcaccggctgggacggccccaccggcctcggaacgccgaacggcaccggagccttcggacaccaccaccaccaccactgaagcttactaggtatctagaaccggtgacgtcaccatgggaagcttcgtggatccagatatccctctagaccgcggccgcccggctgcagcccgtacctctagtagagtcgagggggaacccggccgcgtccggcgcccccgccgccttcgacgagatcccgcaaaagcggcctttgactccctgcaagcctcagcgaccgaatatatcggttatgcgtgggcgatggttgttgtcattgtcggcgcaactatcggtatcaagctgtttaagaaattcacctcgaaagcaagctgataaaccgatacaattaaaggctccttttggagcctttttttttggagattttcaacgtgaaaaaattattattcgcaattcctttagttgttcctttctattctcactccgctgaaactgttgaaagttgtttagcaaaacctcatacagaaaattcatttactaacgtctggaaagacgacaaaactttagatcctctagctagagtcgaccggcatgcaatcgaattcgtaatcatgtcatagctgtttcctgtgtgaaattgttatccgctcacaattccacacaacatacgagccggaagcataaagtgtaaagcctggggtgcctaatgagtgagctaactcacattaattgcgttgcgctcactgcccgctttccagtcgggaaacctgtcgtgccagctgcattaatgaatcggccaacgcgcggggagaggcggtttgcgtattgggcgctcttccgcttcctcgctcactgactcgctgcgctcggtcgttcggctgcggcgagcggtatcagctcactcaaaggcggtaatacggttatccacagaatcaggggataacgcaggaaagaacatgtgagcaaaaggccagcaaaaggccaggaaccgtaaaaaggccgcgttgctggcgtttttccataggctccgcccccctgacgagcatcacaaaaatcgacgctcaagtcagaggtggcgaaacccgacaggactataaagataccaggcgtttccccctggaagctccctcgtgcgctctcctgttccgaccctgccgcttaccggatacctgtccgcctttctcccttcgggaagcgtggcgctttctcatagctcacgctgtaggtatctcagttcggtgtaggtcgttcgctccaagctgggctgtgtgcacgaaccccccgttcagcccgaccgctgcgccttatccggtaactatcgtcttgagtccaacccggtaagacacgacttatcgccactggcagcagccactggtaacaggattagcagagcgaggtatgtaggcggtgctacagagttcttgaagtggtggcctaactacggctacactagaagaacagtatttggtatctgcgctctgctgaagccagttaccttcggaaaaagagttggtagctcttgatccggcaaacaaaccaccgctggtagcggtggtttttttgtttgcaagcagcagattacgcgcagaaaaaaaggatctcaagaagatcctttgatcttttctacggggtctgacgctcagtggaacgaaaactcacgttaagggattttggtcatgagattatcaaaaaggatcttcacctagatccttttggttcatgtgcagctccatcagcaaaaggggatgataagtttatcaccaccgactatttgcaacagtgccgttgatcgtgctatgatcgactgatgtcatcagcggtggagtgcaatgtcgtgcaatacgaatggcgaaaagccgagctcatcggtcagcttctcaaccttggggttacccccggcggtgtgctgctggtccacagctccttccgtagcgtccggcccctcgaagatgggccacttggactgatcgaggccctgcgtgctgcgctgggtccgggagggacgctcgtcatgccctcgtggtcaggtctggacgacgagccgttcgatcctgccacgtcgcccgttacaccggaccttggagttgtctctgacacattctggcgcctgccaaatgtaaagcgcagcgcccatccatttgcctttgcggcagcggggccacaggcagagcagatcatctctgatccattgcccctgccacctcactcgcctgcaagcccggtcgcccgtgtccatgaactcgatgggcaggtacttctcctcggcgtgggacacgatgccaacacgacgctgcatcttgccgagttgatggcaaaggttccctatggggtgccgagacactgcaccattcttcaggatggcaagttggtacgcgtcgattatctcgagaatgaccactgctgtgagcgctttgccttggcggacaggtggctcaaggagaagagccttcagaaggaaggtccagtcggtcatgcctttgctcggttgatccgctcccgcgacattgtggcgacagccctgggtcaactgggccgagatccgttgatcttcctgcatccgccagaggcgggatgcgaagaatgcgatgccgctcgccagtcgattggctgagctcatgagcggagaacgagatgacgttggaggggcaaggtcgcgctgattgctggggcaacacgtggagcggatcggggattgtctttcttcagctcgctgatgatatgctgacgctcaatgccgtttggcctccgactaacgaaaatcccgcatttggacggctgatccgattggcacggcggacggcgaatggcggagcagacgctcgtccgggggcaatgagatatgaaaaagcctgaactcaccgcgacgtatcgggccctggccagctagctagagtcgacctgcaggtccccggggatcggtcttgccttgctcgtcggtgatgtacttcaccagctccgcgaagtcgctcttcttgatggagcgcatggggacgtgcttggcaatcacgcgcaccccccggccgttttagcggctaaaaaagtcatggctctgccctcgggcggaccacgcccatcatgaccttgccaagctcgtcctgcttctcttcgatcttcgccagcagggcgaggatcgtggcatcaccgaaccgcgccgtgcgcgggtcgtcggtgagccagagtttcagcaggccgcccaggcggcccaggtcgccattgatgcgggccagctcgcggacgtgctcatagtccacgacgcccgtgattttgtagccctggccgacggccagcaggtaggccgacaggctcatgccggccgccgccgccttttcctcaatcgctcttcgttcgtctggaaggcagtacaccttgataggtgggctgcccttcctggttggcttggtttcatcagccatccgcttgccctcatctgttacgccggcggtagccggccagcctcgcagagcaggattcccgttgagcaccgccaggtgcgaataagggacagtgaagaaggaacacccgctcgcgggtgggcctacttcacctatcctgcccggctgacgccgttggatacaccaaggaaagtctacacgaaccctttggcaaaatcctgtatatcgtgcgaaaaaggatggatataccgaaaaaatcgctataatgaccccgaagcagggttatgcagcggaaaagatccgtcgacctgcaggcatgc

SEQ ID NO: 29 - DNA, 7518 bp, Unknown
  pMU1s-kasOPSR40gusA
tggcgccggacggggcttcagacgtttcgggtgctgggttgttgtctctggacagtgatccatgggaaactactcagcaccaccaatgttcccaaaagaaagcgcaggtcagcgcccatgagccaagatctaggcatgtcgcccttcatcgctcccgacgtccctgagcaccttctagacactgttcgcgtcttcctgtacgcgcgtcagtctaagggccggtccgacggctcagacgtgtcgaccgaagcacagctagcggccggtcgtgcgttggtcgcgtctcgcaacgcccaggggggtgcgcgctgggtcgtggcaggtgagttcgtggacgtcgggcgctccggctgggacccgaacgtgacccgtgccgacttcgagcgcatgatgggcgaagtccgcgccggcgaaggtgacgttgtcgttgtgaatgagctttcccggctcactcgcaagggcgcccatgacgcgctcgaaatcgacaacgaattgaagaagcacggcgtgcgcttcatgtcggttcttgagccgttccttgacacgtctacccctatcggcgtcgccattttcgcgctgatcgctgcccttgcgaaacaggacagtgacctgaaggcggagcgcctgaagggtgcgaaagacgagattgccgcgctgggtggcgttcactcgtcttccgccccgttcggaatgcgcgccgtgcgcaagaaggtcgataatctcgtgatctccgttcttgagccggacgaagacaacccggatcacgtcgagctagttgagcgcatggcgaaaatgtcgttcgaaggcgtgtccgacaacgccattgcaacgaccttcgagaaggaaaagatcccgtcgcccggaatggctgagagacgcgccacggaaaagcgtcttgcgtccgtcaaggcacgtcgcctgaacggcgctgaaaagccgatcatgtggcgcgctcaaacggtccgatggattctcaaccatcccgcaatcggcggtttcgcattcgagcgtgtgaagcacggtaaggcgcacatcaacgtcatacggcgcgaccccggcggcaagccgctaacgccccacacgggcattctcagcggctcgaagtggcttgagcttcaagagaagcgttccgggaagaatctcagcgaccggaagcctggggccgaagtcgaaccgacgcttctgagcgggtggcgtttcctggggtgccgaatctgcggcggctcaatgggtcagtcccagggtggccgtaagcgcaacggcgaccttgccgaaggcaattacatgtgcgccaacccgaaggggcacggcggcttgtcggtcaagcgcagcgaactggacgaattcgttgcttcgaaggtgtgggcacggctccgcacagccgacatggaagatgaacacgatcaggcatggattgccgccgctgcggagcgcttcgcccttcagcacgacctagcgggggtggccgatgagcggcgcgaacaacaggcgcacctagacaacgtgcggcgctccatcaaggaccttcaggcggaccgtaagcccggtctgtacgtcgggcgtgaagagctggaaacgtggcgctcaacggtgctgcaataccggtcctacgaagcggagtgcacgacccgactcgctgagcttgacgagaagatgaacggcagcacccgcgttccgtctgagtggttcagcggcgaagacccgacggccgaagggggcatctgggcaagctgggacgtgtacgagcgtcgggagttcctgagcttcttccttgactccgtcatggtcgaccgggggcgccaccctgagacgaagaaatacatccccctgaaggaccgtgtgacgctcaagtgggcggagctgctgaaggaggaagacgaagcgagcgaagccactgagcgggagcttgcggcgctgtagcgcacagcgggaggggtcgagccggcggacggttcggccccttttttggccttgaaatcgttagttaggctaactagggtaccgtctctgctttgacaacatgctgtgcggtgttgtaaagtctggtgtaggagaatacgacagcttgtcaaaggagtgtccatatgctgcggcccgtcgaaaccccgacccgcgagatcaagaagctggacggcctgtgggcgttcagcctcgaccgggagaactgcggtatcgaccagcggtggtgggagagcgccctccaggagtcgcgcgccatcgccgtccccggcagcttcaacgaccagttcgcggacgcggacatccgcaactacgcggggaacgtctggtatcagcgggaggtgttcatccccaagggctgggccggtcagcgcatcgtgctgcgcttcgacgccgtgacccactacggcaaggtctgggtcaacaaccaggaagtgatggagcaccagggcggctacacgcccttcgaggcggacgtgaccccgtacgtcatcgccggcaagtcggtccgcatcacggtctgcgtcaacaacgagctcaactggcagaccatcccgcccggcatggtgatcacggacgagaacggcaagaagaagcagagctacttccacgacttcttcaactacgccggcatccaccgctcggtcatgctgtacacgacgccgaacacctgggtcgacgacatcacggtggtcacccacgtggcccaggactgcaaccacgcgtccgtggactggcaggtcgtcgccaacggcgacgtgagcgtggagctccgcgacgccgagcagcaggtcgtggcgaccgggcagggcacctcggggaccctccaggtcgtgaacccccacctctggcagccgggtgagggctacctgtacgagctgtgcgtgacggcgaagagccagaccgagtgcgacatctaccccctgcgcgtcggcatccggtccgtggcggtcaagggcgagcagttcctgatcaaccacaagccgttctacttcacgggcttcggtcggcacgaggacgccgacctccgcggcaagggcttcgacaacgtcctgatggtccacgaccacgccctgatggactggatcggcgccaactcgtaccggacctcgcactacccgtacgcggaagagatgctggactgggcggacgagcacgggatcgtcgtcatcgacgaaaccgccgcggtgggcttcaacctgtccctcggcatcggcttcgaggccggcaacaagccgaaagagctctactccgaagaggccgtcaacggcgaaacccagcaggcccacctccaggcgatcaaagagctcatcgcccgcgacaagaaccacccgtccgtcgtgatgtggtcgatcgccaacgagccggacacccggccgcagggtgcccgggagtacttcgccccgctggccgaggccacccggaagctcgaccccacccggcccatcacctgcgtgaacgtgatgttctgcgacgcccacacggacaccatctccgacctcttcgacgtcctgtgcctgaaccgctactacggctggtacgtgcagtccggggacctggaaacggccgagaaggtcctggagaaagagctgctggcgtggcaggagaagctgcaccagccgatcatcatcaccgagtacggcgtggacacgctggccggtctgcactccatgtacaccgacatgtggtccgaagagtaccagtgcgcgtggctggacatgtaccaccgcgtgttcgaccgcgtcagcgcggtcgtcggcgagcaggtgtggaacttcgccgacttcgccacctcccagggcatcctccgcgtcgggggcaacaagaagggcatcttcacccgggaccgcaagcccaagtcggcggcgttcctgctccagaagcggtggaccgggatgaacttcggggagaagccgcagcagggcgggaagcagtgataagcattacccggatccagatatcctgcaggaattcctcgagccgatatccctctagaccgcggccgcccggctgcagcccgtacctctagtagagtcgagggggaacccggccgcgtccggcgcccccgccgccttcgacgagatcccgcaaaagcggcctttgactccctgcaagcctcagcgaccgaatatatcggttatgcgtgggcgatggttgttgtcattgtcggcgcaactatcggtatcaagctgtttaagaaattcacctcgaaagcaagctgataaaccgatacaattaaaggctccttttggagcctttttttttggagattttcaacgtgaaaaaattattattcgcaattcctttagttgttcctttctattctcactccgctgaaactgttgaaagttgtttagcaaaacctcatacagaaaattcatttactaacgtctggaaagacgacaaaactttagatcctctagctagagtcgaccggcatgcaatcgaattcgtaatcatgtcatagctgtttcctgtgtgaaattgttatccgctcacaattccacacaacatacgagccggaagcataaagtgtaaagcctggggtgcctaatgagtgagctaactcacattaattgcgttgcgctcactgcccgctttccagtcgggaaacctgtcgtgccagctgcattaatgaatcggccaacgcgcggggagaggcggtttgcgtattgggcgctcttccgcttcctcgctcactgactcgctgcgctcggtcgttcggctgcggcgagcggtatcagctcactcaaaggcggtaatacggttatccacagaatcaggggataacgcaggaaagaacatgtgagcaaaaggccagcaaaaggccaggaaccgtaaaaaggccgcgttgctggcgtttttccataggctccgcccccctgacgagcatcacaaaaatcgacgctcaagtcagaggtggcgaaacccgacaggactataaagataccaggcgtttccccctggaagctccctcgtgcgctctcctgttccgaccctgccgcttaccggatacctgtccgcctttctcccttcgggaagcgtggcgctttctcatagctcacgctgtaggtatctcagttcggtgtaggtcgttcgctccaagctgggctgtgtgcacgaaccccccgttcagcccgaccgctgcgccttatccggtaactatcgtcttgagtccaacccggtaagacacgacttatcgccactggcagcagccactggtaacaggattagcagagcgaggtatgtaggcggtgctacagagttcttgaagtggtggcctaactacggctacactagaagaacagtatttggtatctgcgctctgctgaagccagttaccttcggaaaaagagttggtagctcttgatccggcaaacaaaccaccgctggtagcggtggtttttttgtttgcaagcagcagattacgcgcagaaaaaaaggatctcaagaagatcctttgatcttttctacggggtctgacgctcagtggaacgaaaactcacgttaagggattttggtcatgagattatcaaaaaggatcttcacctagatccttttggttcatgtgcagctccatcagcaaaaggggatgataagtttatcaccaccgactatttgcaacagtgccgttgatcgtgctatgatcgactgatgtcatcagcggtggagtgcaatgtcgtgcaatacgaatggcgaaaagccgagctcatcggtcagcttctcaaccttggggttacccccggcggtgtgctgctggtccacagctccttccgtagcgtccggcccctcgaagatgggccacttggactgatcgaggccctgcgtgctgcgctgggtccgggagggacgctcgtcatgccctcgtggtcaggtctggacgacgagccgttcgatcctgccacgtcgcccgttacaccggaccttggagttgtctctgacacattctggcgcctgccaaatgtaaagcgcagcgcccatccatttgcctttgcggcagcggggccacaggcagagcagatcatctctgatccattgcccctgccacctcactcgcctgcaagcccggtcgcccgtgtccatgaactcgatgggcaggtacttctcctcggcgtgggacacgatgccaacacgacgctgcatcttgccgagttgatggcaaaggttccctatggggtgccgagacactgcaccattcttcaggatggcaagttggtacgcgtcgattatctcgagaatgaccactgctgtgagcgctttgccttggcggacaggtggctcaaggagaagagccttcagaaggaaggtccagtcggtcatgcctttgctcggttgatccgctcccgcgacattgtggcgacagccctgggtcaactgggccgagatccgttgatcttcctgcatccgccagaggcgggatgcgaagaatgcgatgccgctcgccagtcgattggctgagctcatgagcggagaacgagatgacgttggaggggcaaggtcgcgctgattgctggggcaacacgtggagcggatcggggattgtctttcttcagctcgctgatgatatgctgacgctcaatgccgtttggcctccgactaacgaaaatcccgcatttggacggctgatccgattggcacggcggacggcgaatggcggagcagacgctcgtccgggggcaatgagatatgaaaaagcctgaactcaccgcgacgtatcgggccctggccagctagctagagtcgacctgcaggtccccggggatcggtcttgccttgctcgtcggtgatgtacttcaccagctccgcgaagtcgctcttcttgatggagcgcatggggacgtgcttggcaatcacgcgcaccccccggccgttttagcggctaaaaaagtcatggctctgccctcgggcggaccacgcccatcatgaccttgccaagctcgtcctgcttctcttcgatcttcgccagcagggcgaggatcgtggcatcaccgaaccgcgccgtgcgcgggtcgtcggtgagccagagtttcagcaggccgcccaggcggcccaggtcgccattgatgcgggccagctcgcggacgtgctcatagtccacgacgcccgtgattttgtagccctggccgacggccagcaggtaggccgacaggctcatgccggccgccgccgccttttcctcaatcgctcttcgttcgtctggaaggcagtacaccttgataggtgggctgcccttcctggttggcttggtttcatcagccatccgcttgccctcatctgttacgccggcggtagccggccagcctcgcagagcaggattcccgttgagcaccgccaggtgcgaataagggacagtgaagaaggaacacccgctcgcgggtgggcctacttcacctatcctgcccggctgacgccgttggatacaccaaggaaagtctacacgaaccctttggcaaaatcctgtatatcgtgcgaaaaaggatggatataccgaaaaaatcgctataatgaccccgaagcagggttatgcagcggaaaagatccgtcgacctgcaggcatgc

SEQ ID NO: 30 - DNA, 38 bp, Unknown
  ermEp1* promoter
gttgtgggcacaatcgtgccggttggtaggatccagcg